European Patent Specification EP 3 835 310 B1, published March 20, 2024. Title: FIBRONECTIN BASED SCAFFOLD DOMAIN PROTEINS THAT BIND TO MYOSTATIN. Applicant: BRISTOL-MYERS SQUIBB COMPANY. Application EP. The sequence listing filed with the application follows.

SEQUENCE LISTING (331 sequences)

SEQ ID NO: 1 - protein, 375 aa, Homo sapiens
MQKLQLCVYIYLFMLIVAGPVDLNENSEQKENVEKEGLCNACTWRQNTKSSRIEAIKIQILSKLRLETAPNISKDVIRQLLPKAPPLRELIDQYDVQRDDSSDGSLEDDDYHATTETIITMPTESDFLMQVDGKPKCCFFKFSSKIQYNKVVKAQLWIYLRPVETPTTVFVQILRLIKPMKDGTRYTGIRSLKLDMNPGTGIWQSIDVKTVLQNWLKQPESNLGIEIKALDENGHDLAVTFPGPGEDGLNPFLEVKVTDTPKRSRRDFGLDCDEHSTESRCCRYPLTVDFEAFGWDWIIAPKRYKANYCSGECEFVFLQKYPHTHLVHQANPRGSAGPCCTPTKMSPINMLYFNGKEQIIYGKIPAMVVDRCGCS

SEQ ID NO: 2 - protein, 352 aa, Homo sapiens [sequence omitted]

SEQ ID NO: 3 - protein, 109 aa, Homo sapiens
DFGLDCDEHSTESRCCRYPLTVDFEAFGWDWIIAPKRYKANYCSGECEFVFLQKYPHTHLVHQANPRGSAGPCCTPTKMSPINMLYFNGKEQIIYGKIPAMVVDRCGCS

SEQ ID NO: 4 - protein, 94 aa, Homo sapiens
VSDVPRDLEVVAATPTSLLISWDAPAVTVRYYRITYGETGGNSPVQEFTVPGSKSTATISGLKPGVDYTITVYAVTGRGDSPASSKPISINYRT

SEQ ID NO: 5 - protein, 157 aa, Artificial Sequence
  Synthetic
  misc_feature (7)..(21): Xaa, if present, can be any naturally occurring amino acid
  misc_feature (26)..(45): Xaa, if present, can be any naturally occurring amino acid
  misc_feature (54)..(73): Xaa, if present, can be any naturally occurring amino acid
  misc_feature (79)..(98): Xaa, if present, can be any naturally occurring amino acid
  misc_feature (102)..(121): Xaa, if present, can be any naturally occurring amino acid
  misc_feature (131)..(150): Xaa, if present, can be any naturally occurring amino acid
EVVAATXXXXXXXXXXXXXXXSLLIXXXXXXXXXXXXXXXXXXXXYYRITYGEXXXXXXXXXXXXXXXXXXXXQEFTVXXXXXXXXXXXXXXXXXXXXATIXXXXXXXXXXXXXXXXXXXXDYTITVYAVXXXXXXXXXXXXXXXXXXXXISINYRT

SEQ ID NO: 6 - protein, 118 aa, Artificial Sequence
  Synthetic
  misc_feature (13)..(32): Xaa, if present, can be any naturally occurring amino acid
  misc_feature (53)..(72): Xaa, if present, can be any naturally occurring amino acid
  misc_feature (92)..(111): Xaa, if present, can be any naturally occurring amino acid
EVVAATPTSLLIXXXXXXXXXXXXXXXXXXXXYYRITYGETGGNSPVQEFTVXXXXXXXXXXXXXXXXXXXXATISGLKPGVDYTITVYAVXXXXXXXXXXXXXXXXXXXXISINYRT

SEQ ID NO: 7 - protein, 11 aa, Artificial Sequence
  Synthetic
SWSLPHAGHVN

SEQ ID NO: 8 - protein, 10 aa, Artificial Sequence
  Synthetic
SWVSPRGRAR

SEQ ID NO: 9 - protein, 10 aa, Artificial Sequence
  Synthetic
SWEVPRGLAR

SEQ ID NO: 10 - protein, 10 aa, Artificial Sequence
  Synthetic
SWWAPLGLAR

SEQ ID NO: 11 - protein, 11 aa, Artificial Sequence
  Synthetic
SWTLPHAGLAH

SEQ ID NO: 12 - protein, 11 aa, Artificial Sequence
  Synthetic
SWYLPYPAHMN

SEQ ID NO: 13 - protein, 11 aa, Artificial Sequence
  Synthetic
SWSLPFAGHLN

SEQ ID NO: 14 - protein, 11 aa, Artificial Sequence
  Synthetic
SWSLPYSGLAN

SEQ ID NO: 15 - protein, 11 aa, Artificial Sequence
  Synthetic
SWSLPHAGHAH

SEQ ID NO: 16 - protein, 11 aa, Artificial Sequence
  Synthetic
SWTLPNFGLIN

SEQ ID NO: 17 - protein, 11 aa, Artificial Sequence
  Synthetic
SWTLPHAGRAH

SEQ ID NO: 18 - protein, 11 aa, Artificial Sequence
  Synthetic
SWSLPYAGHLN

SEQ ID NO: 19 - protein, 11 aa, Artificial Sequence
  Synthetic
SWSLPYAAHMN

SEQ ID NO: 20 - protein, 11 aa, Artificial Sequence
  Synthetic
SWSLPYPGHLN

SEQ ID NO: 21 - protein, 11 aa, Artificial Sequence
  Synthetic
SWSLPYAGHAH

SEQ ID NO: 22 - protein, 10 aa, Artificial Sequence
  Synthetic
SWDAPGGLAR

SEQ ID NO: 23 - protein, 11 aa, Artificial Sequence
  Synthetic
SWSLPTPGLAH

SEQ ID NO: 24 - protein, 11 aa, Artificial Sequence
  Synthetic
SWSLPHRGVAN

SEQ ID NO: 25 - protein, 11 aa, Artificial Sequence
  Synthetic
SWSLPSSGVAH

SEQ ID NO: 26 - protein, 11 aa, Artificial Sequence
  Synthetic
SWSLPHHGFGH

SEQ ID NO: 27 - protein, 11 aa, Artificial Sequence
  Synthetic
SWSLPHAGDAH

SEQ ID NO: 28 - protein, 11 aa, Artificial Sequence
  Synthetic
SWSLPHNGVAH

SEQ ID NO: 29 - protein, 11 aa, Artificial Sequence
  Synthetic
SWSLPRQGLAN

SEQ ID NO: 30 - protein, 11 aa, Artificial Sequence
  Synthetic
SWSLPGPGHFH

SEQ ID NO: 31 - protein, 11 aa, Artificial Sequence
  Synthetic
SWSLPHPGLGH

SEQ ID NO: 32 - protein, 10 aa, Artificial Sequence
  Synthetic
SWDAPRGLAR

SEQ ID NO: 33 - protein, 10 aa, Artificial Sequence
  Synthetic
SWDAPAGLAR

SEQ ID NO: 34 - protein, 11 aa, Artificial Sequence
  Synthetic
SWSLPHQGKAN

SEQ ID NO: 35 - protein, 10 aa, Artificial Sequence
  Synthetic
SWDAPKGLAR

SEQ ID NO: 36 - protein, 11 aa, Artificial Sequence
  Synthetic
SWSLPNPGIAH

SEQ ID NO: 37 - protein, 11 aa, Artificial Sequence
  Synthetic
SWSLPRPGNAH

SEQ ID NO: 38 - protein, 11 aa, Artificial Sequence
  Synthetic
SWSLPNPGNAH

SEQ ID NO: 39 - protein, 6 aa, Artificial Sequence
  Synthetic
PGRGVT

SEQ ID NO: 40 - protein, 6 aa, Artificial Sequence
  Synthetic
PGRGST

SEQ ID NO: 41 - protein, 6 aa, Artificial Sequence
  Synthetic
LGRGST

SEQ ID NO: 42 - protein, 6 aa, Artificial Sequence
  Synthetic
PGRGLT

SEQ ID NO: 43 - protein, 6 aa, Artificial Sequence
  Synthetic
IGRGST

SEQ ID NO: 44 - protein, 6 aa, Artificial Sequence
  Synthetic
FGRGTT

SEQ ID NO: 45 - protein, 6 aa, Artificial Sequence
  Synthetic
VGRGNT

SEQ ID NO: 46 - protein, 12 aa, Artificial Sequence
  Synthetic
TLTKSQMIHYMP

SEQ ID NO: 47 - protein, 12 aa, Artificial Sequence
  Synthetic
TIYRDGMSHHDP

SEQ ID NO: 48 - protein, 12 aa, Artificial Sequence
  Synthetic
TVYRDGPLLLAP

SEQ ID NO: 49 - protein, 12 aa, Artificial Sequence
  Synthetic
TIFRTGMVQYDP

SEQ ID NO: 50 - protein, 12 aa, Artificial Sequence
  Synthetic
TLTNSEIILYKP

SEQ ID NO: 51 - protein, 12 aa, Artificial Sequence
  Synthetic
TLTKSQILHHRP

SEQ ID NO: 52 - protein, 12 aa, Artificial Sequence
  Synthetic
TLTRSKIIHYMP

SEQ ID NO: 53 - protein, 12 aa, Artificial Sequence
  Synthetic
TLTHSNIIRYVP

SEQ ID NO: 54 - protein, 12 aa, Artificial Sequence
  Synthetic
TVSSTKVIVYLP

SEQ ID NO: 55 - protein, 12 aa, Artificial Sequence
  Synthetic
TITKSTIIIYKP

SEQ ID NO: 56 - protein, 12 aa, Artificial Sequence
  Synthetic
TVTTTSVILYKP

SEQ ID NO: 57 - protein, 12 aa, Artificial Sequence
  Synthetic
TLTKSQLIHYMP

SEQ ID NO: 58 - protein, 12 aa, Artificial Sequence
  Synthetic
TLTRSQVIHYMP

SEQ ID NO: 59 - protein, 12 aa, Artificial Sequence
  Synthetic
TLTKSKIIHYMP

SEQ ID NO: 60 - protein, 12 aa, Artificial Sequence
  Synthetic
TVSSTKVIHYKP

SEQ ID NO: 61 - protein, 12 aa, Artificial Sequence
  Synthetic
TLTKSKVIHYMP

SEQ ID NO: 62 - protein, 12 aa, Artificial Sequence
  Synthetic
TVTTTKVIHYKP

SEQ ID NO: 63 - protein, 12 aa, Artificial Sequence
  Synthetic
TIDRDGVNHFAP

SEQ ID NO: 64 - protein, 12 aa, Artificial Sequence
  Synthetic
TVTHHGVIGYKP

SEQ ID NO: 65 - protein, 12 aa, Artificial Sequence
  Synthetic
TLTGANVIIYKP

SEQ ID NO: 66 - protein, 12 aa, Artificial Sequence
  Synthetic
TVTNTGVIIYKP

SEQ ID NO: 67 - protein, 12 aa, Artificial Sequence
  Synthetic
TVTATGIIIYKP

SEQ ID NO: 68 - protein, 12 aa, Artificial Sequence
  Synthetic
TVTRAGFYRYKP

SEQ ID NO: 69 - protein, 12 aa, Artificial Sequence
  Synthetic
TVTREEVISYKP

SEQ ID NO: 70 - protein, 12 aa, Artificial Sequence
  Synthetic
TVTAAGVIIYKP

SEQ ID NO: 71 - protein, 12 aa, Artificial Sequence
  Synthetic
TVTANQPIIYKP

SEQ ID NO: 72 - protein, 12 aa, Artificial Sequence
  Synthetic
TITPETIIVYKP

SEQ ID NO: 73 - protein, 12 aa, Artificial Sequence
  Synthetic
TIDRDGTRSFDP

SEQ ID NO: 74 - protein, 12 aa, Artificial Sequence
  Synthetic
TIFRDGPVTWDP

SEQ ID NO: 75 - protein, 12 aa, Artificial Sequence
  Synthetic
TVTDTGYLKYKP

SEQ ID NO: 76 - protein, 12 aa, Artificial Sequence
  Synthetic
TLTGSDTIFYKP

SEQ ID NO: 77 - protein, 12 aa, Artificial Sequence
  Synthetic
TVTGKDVIKYKP

SEQ ID NO: 78 - protein, 12 aa, Artificial Sequence
  Synthetic
TIFRDGVVNYGP

SEQ ID NO: 79 - protein, 12 aa, Artificial Sequence
  Synthetic
TVTDTGFITYKP

SEQ ID NO: 80 - protein, 110 aa, Artificial Sequence
  Synthetic
MGVSDVPRDLEVVAATPTSLLISWSLPHAGHVNYYRITYGETGGNSPVQEFTVPGRGVTATISGLKPGVDYTITVYAVTLTKSQMIHYMPISINYRTEIDKPSQHHHHHH

SEQ ID NO: 81 - protein, 109 aa, Artificial Sequence
  Synthetic
MGVSDVPRDLEVVAATPTSLLISWVSPRGRARYYRITYGETGGNSPVQEFTVPGRGSTATISGLKPGVDYTITVYAVTIYRDGMSHHDPISINYRTEIDKPSQHHHHHH

SEQ ID NO: 82 - protein, 109 aa, Artificial Sequence
  Synthetic
MGVSDVPRDLEVVAATPTSLLISWEVPRGLARYYRITYGETGGNSPVQEFTVLGRGSTATISGLKPGVDYTITVYAVTVYRDGPLLLAPISINYRTEIDKPSQHHHHHH

SEQ ID NO: 83 - protein, 109 aa, Artificial Sequence
  Synthetic
MGVSDVPRDLEVVAATPTSLLISWWAPLGLARYYRITYGETGGNSPVQEFTVPGRGSTATISGLKPGVDYTITVYAVTIFRTGMVQYDPISINYRTEIDKPSQHHHHHH

SEQ ID NO: 84 - protein, 110 aa, Artificial Sequence
  Synthetic
MGVSDVPRDLEVVAATPTSLLISWTLPHAGLAHYYRITYGETGGNSPVQEFTVPGRGVTATISGLKPGVDYTITVYAVTLTNSEIILYKPISINYRTEIDKPSQHHHHHH

SEQ ID NO: 85 - protein, 110 aa, Artificial Sequence
  Synthetic
MGVSDVPRDLEVVAATPTSLLISWYLPYPAHMNYYRITYGETGGNSPVQEFTVPGRGLTATISGLKPGVDYTITVYAVTLTKSQILHHRPISINYRTEIDKPSQHHHHHH

SEQ ID NO: 86 - protein, 110 aa, Artificial Sequence
  Synthetic
MGVSDVPRDLEVVAATPTSLLISWSLPFAGHLNYYRITYGETGGNSPVQEFTVPGRGVTATISGLKPGVDYTITVYAVTLTRSKIIHYMPISINYRTEIDKPSQHHHHHH

SEQ ID NO: 87 - protein, 110 aa, Artificial Sequence
  Synthetic
MGVSDVPRDLEVVAATPTSLLISWSLPYSGLANYYRITYGETGGNSPVQEFTVPGRGVTATISGLKPGVDYTITVYAVTLTHSNIIRYVPISINYRTEIDKPSQHHHHHH

SEQ ID NO: 88 - protein, 110 aa, Artificial Sequence
  Synthetic
MGVSDVPRDLEVVAATPTSLLISWSLPHAGHAHYYRITYGETGGNSPVQEFTVPGRGVTATISGLKPGVDYTITVYAVTVSSTKVIVYLPISINYRTEIDKPSQHHHHHH

SEQ ID NO: 89 - protein, 110 aa, Artificial Sequence
  Synthetic
MGVSDVPRDLEVVAATPTSLLISWTLPNFGLINYYRITYGETGGNSPVQEFTVPGRGVTATISGLKPGVDYTITVYAVTITKSTIIIYKPISINYRTEIDKPSQHHHHHH

SEQ ID NO: 90 - protein, 110 aa, Artificial Sequence
  Synthetic
MGVSDVPRDLEVVAATPTSLLISWTLPHAGRAHYYRITYGETGGNSPVQEFTVPGRGVTATISGLKPGVDYTITVYAVTVTTTSVILYKPISINYRTEIDKPSQHHHHHH

SEQ ID NO: 91 - protein, 110 aa, Artificial Sequence
  Synthetic
MGVSDVPRDLEVVAATPTSLLISWSLPYAGHLNYYRITYGETGGNSPVQEFTVPGRGVTATISGLKPGVDYTITVYAVTLTKSQLIHYMPISINYRTEIDKPSQHHHHHH

SEQ ID NO: 92 - protein, 110 aa, Artificial Sequence
  Synthetic
MGVSDVPRDLEVVAATPTSLLISWSLPYAAHMNYYRITYGETGGNSPVQEFTVPGRGVTATISGLKPGVDYTITVYAVTLTRSQVIHYMPISINYRTEIDKPSQHHHHHH

SEQ ID NO: 93 - protein, 110 aa, Artificial Sequence
  Synthetic
MGVSDVPRDLEVVAATPTSLLISWSLPHAGHAHYYRITYGETGGNSPVQEFTVPGRGVTATISGLKPGVDYTITVYAVTLTKSKIIHYMPISINYRTEIDKPSQHHHHHH

SEQ ID NO: 94 - protein, 110 aa, Artificial Sequence
  Synthetic
MGVSDVPRDLEVVAATPTSLLISWSLPYPGHLNYYRITYGETGGNSPVQEFTVPGRGVTATISGLKPGVDYTITVYAVTLTKSKIIHYMPISINYRTEIDKPSQHHHHHH

SEQ ID NO: 95 - protein, 110 aa, Artificial Sequence
  Synthetic
MGVSDVPRDLEVVAATPTSLLISWTLPHAGRAHYYRITYGETGGNSPVQEFTVPGRGVTATISGLKPGVDYTITVYAVTLTRSKIIHYMPISINYRTEIDKPSQHHHHHH

SEQ ID NO: 96 - protein, 110 aa, Artificial Sequence
  Synthetic
MGVSDVPRDLEVVAATPTSLLISWSLPYAGHAHYYRITYGETGGNSPVQEFTVPGRGVTATISGLKPGVDYTITVYAVTLTKSKIIHYMPISINYRTEIDKPSQHHHHHH

SEQ ID NO: 97 - protein, 110 aa, Artificial Sequence
  Synthetic
MGVSDVPRDLEVVAATPTSLLISWSLPHAGHAHYYRITYGETGGNSPVQEFTVPGRGVTATISGLKPGVDYTITVYAVTLTRSKIIHYMPISINYRTEIDKPSQHHHHHH

SEQ ID NO: 98 - protein, 110 aa, Artificial Sequence
  Synthetic
MGVSDVPRDLEVVAATPTSLLISWSLPYPGHLNYYRITYGETGGNSPVQEFTVPGRGVTATISGLKPGVDYTITVYAVTLTRSKIIHYMPISINYRTEIDKPSQHHHHHH

SEQ ID NO: 99 - protein, 110 aa, Artificial Sequence
  Synthetic
MGVSDVPRDLEVVAATPTSLLISWTLPHAGRAHYYRITYGETGGNSPVQEFTVPGRGVTATISGLKPGVDYTITVYAVTVSSTKVIHYKPISINYRTEIDKPSQHHHHHH

SEQ ID NO: 100 - protein, 110 aa, Artificial Sequence
  Synthetic
MGVSDVPRDLEVVAATPTSLLISWSLPYAGHAHYYRITYGETGGNSPVQEFTVPGRGVTATISGLKPGVDYTITVYAVTLTRSKIIHYMPISINYRTEIDKPSQHHHHHH

SEQ ID NO: 101 - protein, 110 aa, Artificial Sequence
  Synthetic
MGVSDVPRDLEVVAATPTSLLISWSLPHAGHAHYYRITYGETGGNSPVQEFTVPGRGVTATISGLKPGVDYTITVYAVTLTKSKVIHYMPISINYRTEIDKPSQHHHHHH

SEQ ID NO: 102 - protein, 110 aa, Artificial Sequence
  Synthetic
MGVSDVPRDLEVVAATPTSLLISWSLPYPGHLNYYRITYGETGGNSPVQEFTVPGRGVTATISGLKPGVDYTITVYAVTLTKSKVIHYMPISINYRTEIDKPSQHHHHHH

SEQ ID NO: 103 - protein, 110 aa, Artificial Sequence
  Synthetic
MGVSDVPRDLEVVAATPTSLLISWTLPHAGRAHYYRITYGETGGNSPVQEFTVPGRGVTATISGLKPGVDYTITVYAVTVSSTKVIVYLPISINYRTEIDKPSQHHHHHH

SEQ ID NO: 104 - protein, 110 aa, Artificial Sequence
  Synthetic
MGVSDVPRDLEVVAATPTSLLISWSLPYAGHAHYYRITYGETGGNSPVQEFTVPGRGVTATISGLKPGVDYTITVYAVTLTKSKVIHYMPISINYRTEIDKPSQHHHHHH

SEQ ID NO: 105 - protein, 110 aa, Artificial Sequence
  Synthetic
MGVSDVPRDLEVVAATPTSLLISWTLPHAGRAHYYRITYGETGGNSPVQEFTVPGRGVTATISGLKPGVDYTITVYAVTVTTTKVIHYKPISINYRTEIDKPSQHHHHHH

SEQ ID NO: 106 - protein, 109 aa, Artificial Sequence
  Synthetic
MGVSDVPRDLEVVAATPTSLLISWDAPGGLARYYRITYGETGGNSPVQEFTVIGRGSTATISGLKPGVDYTITVYAVTIDRDGVNHFAPISINYRTEIDKPSQHHHHHH

SEQ ID NO: 107 - protein, 110 aa, Artificial Sequence
  Synthetic
MGVSDVPRDLEVVAATPTSLLISWSLPTPGLAHYYRITYGETGGNSPVQEFTVPGRGVTATISGLKPGVDYTITVYAVTVTHHGVIGYKPISINYRTEIDKPSQHHHHHH

SEQ ID NO: 108 - protein, 110 aa, Artificial Sequence
  Synthetic
MGVSDVPRDLEVVAATPTSLLISWSLPHRGVANYYRITYGETGGNSPVQEFTVPGRGVTATISGLKPGVDYTITVYAVTLTGANVIIYKPISINYRTEIDKPSQHHHHHH

SEQ ID NO: 109 - protein, 110 aa, Artificial Sequence
  Synthetic
MGVSDVPRDLEVVAATPTSLLISWSLPSSGVAHYYRITYGETGGNSPVQEFTVPGRGVTATISGLKPGVDYTITVYAVTVTNTGVIIYKPISINYRTEIDKPSQHHHHHH

SEQ ID NO: 110 - protein, 110 aa, Artificial Sequence
  Synthetic
MGVSDVPRDLEVVAATPTSLLISWSLPHHGFGHYYRITYGETGGNSPVQEFTVPGRGVTATISGLKPGVDYTITVYAVTVTATGIIIYKPISINYRTEIDKPSQHHHHHH

SEQ ID NO: 111 - protein, 110 aa, Artificial Sequence
  Synthetic
MGVSDVPRDLEVVAATPTSLLISWSLPHAGDAHYYRITYGETGGNSPVQEFTVPGRGVTATISGLKPGVDYTITVYAVTVTRAGFYRYKPISINYRTEIDKPSQHHHHHH

SEQ ID NO: 112 - protein, 110 aa, Artificial Sequence
  Synthetic
MGVSDVPRDLEVVAATPTSLLISWSLPHNGVAHYYRITYGETGGNSPVQEFTVPGRGVTATISGLKPGVDYTITVYAVTVTREEVISYKPISINYRTEIDKPSQHHHHHH

SEQ ID NO: 113 - protein, 110 aa, Artificial Sequence
  Synthetic
MGVSDVPRDLEVVAATPTSLLISWSLPRQGLANYYRITYGETGGNSPVQEFTVPGRGVTATISGLKPGVDYTITVYAVTVTAAGVIIYKPISINYRTEIDKPSQHHHHHH

SEQ ID NO: 114 - protein, 110 aa, Artificial Sequence
  Synthetic
MGVSDVPRDLEVVAATPTSLLISWSLPGPGHFHYYRITYGETGGNSPVQEFTVPGRGVTATISGLKPGVDYTITVYAVTVTANQPIIYKPISINYRTEIDKPSQHHHHHH

SEQ ID NO: 115 - protein, 110 aa, Artificial Sequence
  Synthetic
MGVSDVPRDLEVVAATPTSLLISWSLPHPGLGHYYRITYGETGGNSPVQEFTVPGRGVTATISGLKPGVDYTITVYAVTITPETIIVYKPISINYRTEIDKPSQHHHHHH

SEQ ID NO: 116 - protein, 109 aa, Artificial Sequence
  Synthetic
MGVSDVPRDLEVVAATPTSLLISWDAPRGLARYYRITYGETGGNSPVQEFTVFGRGTTATISGLKPGVDYTITVYAVTIDRDGTRSFDPISINYRTEIDKPSQHHHHHH

SEQ ID NO: 117 - protein, 109 aa, Artificial Sequence
  Synthetic
MGVSDVPRDLEVVAATPTSLLISWDAPAGLARYYRITYGETGGNSPVQEFTVVGRGNTATISGLKPGVDYTITVYAVTIFRDGPVTWDPISINYRTEIDKPSQHHHHHH

SEQ ID NO: 118 - protein, 110 aa, Artificial Sequence
  Synthetic
MGVSDVPRDLEVVAATPTSLLISWSLPHQGKANYYRITYGETGGNSPVQEFTVPGRGVTATISGLKPGVDYTITVYAVTVTDTGYLKYKPISINYRTEIDKPSQHHHHHH

SEQ ID NO: 119 - protein, 109 aa, Artificial Sequence
  Synthetic
MGVSDVPRDLEVVAATPTSLLISWDAPKGLARYYRITYGETGGNSPVQEFTVVGRGNTATISGLKPGVDYTITVYAVTIFRDGPVTWDPISINYRTEIDKPSQHHHHHH

SEQ ID NO: 120 - protein, 110 aa, Artificial Sequence
  Synthetic
MGVSDVPRDLEVVAATPTSLLISWSLPNPGIAHYYRITYGETGGNSPVQEFTVPGRGVTATISGLKPGVDYTITVYAVTLTGSDTIFYKPISINYRTEIDKPSQHHHHHH

SEQ ID NO: 121 - protein, 110 aa, Artificial Sequence
  Synthetic
MGVSDVPRDLEVVAATPTSLLISWSLPRPGNAHYYRITYGETGGNSPVQEFTVPGRGVTATISGLKPGVDYTITVYAVTVTGKDVIKYKPISINYRTEIDKPSQHHHHHH

SEQ ID NO: 122 - protein, 109 aa, Artificial Sequence
  Synthetic
MGVSDVPRDLEVVAATPTSLLISWDAPAGLARYYRITYGETGGNSPVQEFTVVGRGNTATISGLKPGVDYTITVYAVTIFRDGVVNYGPISINYRTEIDKPSQHHHHHH

SEQ ID NO: 123 - protein, 110 aa, Artificial Sequence
  Synthetic
MGVSDVPRDLEVVAATPTSLLISWSLPNPGNAHYYRITYGETGGNSPVQEFTVPGRGVTATISGLKPGVDYTITVYAVTVTDTGFITYKPISINYRTEIDKPSQHHHHHH

SEQ ID NO: 124 - DNA, 330 bp, Artificial Sequence
  Synthetic
atgggagtttctgatgtgccgcgcgacctggaagtggttgctgccacccccaccagcctgctgatcagctggtctctgccgcatgctggtcatgtgaactattaccgcatcacttacggcgaaacaggaggcaatagccctgtccaggagttcactgtgcctggtcgtggtgttacagctaccatcagcggccttaaacctggcgttgattataccatcactgtgtatgctgtcactctgactaaatctcagatgatccattacatgccaatttccattaattaccgcacagaaattgacaaaccatcccagcaccatcaccaccaccac

SEQ ID NO: 125 - DNA, 327 bp, Artificial Sequence
  Synthetic
atgggagtttctgatgtgccgcgcgacctggaagtggttgctgccacccccaccagcctgctgatcagctgggtttctccgcgtggtcgtgctcgatattaccgcatcacttacggcgaaacaggaggcaatagccctgtccaggagttcactgtgcctggtcgtggttctacagctaccatcagcggccttaaacctggcgttgattataccatcactgtgtatgctgtcactatctaccgtgacggtatgtctcatcatgacccaatttccattaattaccgcacagaaattgacaaaccatcccagcaccatcaccaccaccac

SEQ ID NO: 126 - DNA, 327 bp, Artificial Sequence
  Synthetic
atgggagtttctgatgtgccgcgcgacctggaagtggttgctgccacccccaccagcctgctgatcagctgggaagtgccgcgtggcctagctcgatattaccgcatcacttacggcgaaacaggaggcaatagccctgtccaggagttcactgtgcttggtcgtggttctacagctaccatcagcggccttaaacctggcgttgattataccatcactgtgtatgctgtcactgtgtaccgtgacgggccgttgcttcttgccccaatttccattaattaccgcacagaaattgacaaaccatcccagcaccatcaccaccaccac

SEQ ID NO: 127 - DNA, 327 bp, Artificial Sequence
  Synthetic
atgggagtttctgatgtgccgcgcgacctggaagtggttgctgccacccccaccagcctgctgatcagctggtgggccccgctgggtcttgctcgatattaccgcatcacttacggcgaaacaggaggcaatagccctgtccaggagttcactgtgcctggtcggggctctacagctaccatcagcggccttaaacctggcgttgattataccatcactgtgtatgctgtcactatcttccgtacgggcatggttcaatatgacccaatttccattaattaccgcacagaaattgacaaaccatcccagcaccatcaccaccaccac

SEQ ID NO: 128 - DNA, 330 bp, Artificial Sequence
  Synthetic
atgggagtttctgatgtgccgcgcgacctggaagtggttgctgccacccccaccagcctgctgatcagctggactctgccgcatgctggtcttgcgcactattaccgcatcacttacggcgaaacaggaggcaatagccctgtccaggagttcactgtgcctggtcgtggtgttacagctaccatcagcggccttaaacctggcgttgattataccatcactgtgtatgctgtcactctgactaattctgagattatcctttacaagccaatttccattaattaccgcacagaaattgacaaaccatcccagcaccatcaccaccaccac

SEQ ID NO: 129 - DNA, 330 bp, Artificial Sequence
  Synthetic
atgggagtttctgatgtgccgcgcgacctggaagtggttgctgccacccccaccagcctgctgatcagctggtacctcccgtatcctgcgcatatgaactattaccgcatcacttacggcgaaacaggaggcaatagccctgtccaggagttcactgtgcctgggcggggtctgacagctaccatcagcggccttaaacctggcgttgattataccatcactgtgtatgctgtcactctgacaaaatctcagattctccatcataggccaatttccattaattaccgcacagaaattgacaaaccatcccagcaccatcaccaccaccac

SEQ ID NO: 130 - DNA, 330 bp, Artificial Sequence
  Synthetic
atgggagtttctgatgtgccgcgcgacctggaagtggttgctgccacccccaccagcctgctgatcagctggtcattgccgtttgctggtcatttgaactattaccgcatcacttacggcgaaacaggaggcaatagccctgtccaggagttcactgtgcctggtcgtggtgttacagctaccatcagcggccttaaacctggcgttgattataccatcactgtgtatgctgtcactctgactcgctctaagattattcattatatgccaatttccattaattaccgcacagaaattgacaaaccatcccagcaccatcaccaccaccac

SEQ ID NO: 131 - DNA, 330 bp, Artificial Sequence
  Synthetic
atgggagtttctgatgtgccgcgcgacctggaagtggttgctgccacccccaccagcctgctgatcagctggtctctgccttattctggccttgcgaactattaccgcatcacttacggcgaaacaggaggcaatagccctgtccaggagttcactgtgcctggtcgtggggttacagctactatcagcggccttaaacctggcgttgattataccatcactgtgtatgctgtcactctgactcactctaatataattcgatacgtgccaatttccattaattaccgcacagaaattgacaaaccatcccagcaccatcaccaccaccac

SEQ ID NO: 132 - DNA, 330 bp, Artificial Sequence
  Synthetic
atgggagtttctgatgtgccgcgcgacctggaagtggttgctgccacccccaccagcctgctgatcagctggtccctaccgcatgcgggtcatgcgcactattaccgcatcacttacggcgaaacaggaggcaatagccctgtccaggagttcactgtgcctggtcgtggagttacagctaccatcagcggccttaaacctggcgttgattataccatcactgtgtatgctgtcactgtgtctagtacaaaggtgatagtttacctgccaatttccattaattaccgcacagaaattgacaaaccatcccagcaccatcaccaccaccac

SEQ ID NO: 133 - DNA, 330 bp, Artificial Sequence
  Synthetic
atgggagtttctgatgtgccgcgcgacctggaagtggttgctgccacccccaccagcctgctgatcagctggactttgccgaatttcggtcttattaattattaccgcatcacttacggcgaaacaggaggcaatagccctgtccaggagttcactgtgcctggtcgtggtgttacagctaccatcagcggccttaaacctggcgttgattataccatcactgtgtatgctgtcactatcaccaaatctactatcatcatttacaagccaatttccattaattaccgcacagaaattgacaaaccatcccagcaccatcaccaccaccac

SEQ ID NO: 134 - DNA, 330 bp, Artificial Sequence
  Synthetic
atgggagtttctgatgtgccgcgcgacctggaagtggttgctgccacccccaccagcctgctgatcagctggactttgccgcatgctggtcgtgcgcactattaccgcatcacttacggcgaaacaggaggcaatagccctgtccaggagttcactgtgcctgggcggggtgttacagctaccatcagcggccttaaacctggcgttgattataccatcactgtgtatgctgtcactgtgacgacaacttcggtgatcctttacaagccaatttccattaattaccgcacagaaattgacaaaccatcccagcaccatcaccaccaccac

SEQ ID NO: 135 - DNA, 330 bp, Artificial Sequence
  Synthetic
atgggagtttctgatgtgccgcgcgacctggaagtggttgctgccacccccaccagcctgctgatcagctggtctcttccttatgctggtcatctaaactattaccgcatcacttacggcgaaacaggaggcaatagccctgtccaggagttcactgtgcctggtcgtggtgtgacagctaccatcagcggccttaaacctggcgttgattataccatcactgtgtatgctgtcactctgactaagtctcagctgatacattacatgccaatttccattaattaccgcacagaaattgacaaaccatcccagcaccatcaccaccaccac

SEQ ID NO: 136 - DNA, 330 bp, Artificial Sequence
  Synthetic
atgggagtttctgatgtgccgcgcgacctggaagtggttgctgccacccccaccagcctgctgatcagctggtctctgccgtatgctgctcacatgaactattaccgcatcacttacggcgaaacaggaggcaatagccctgtccaggagttcactgtgcctggtcgtggtgttacagctaccatcagcggccttaaacctggcgttgattataccatcactgtgtatgctgtcactttgactagatcacaggtgattcattacatgccaatttccattaattaccgcacagaaattgacaaaccatcccagcaccatcaccaccaccac

SEQ ID NO: 137 - DNA, 330 bp, Artificial Sequence
  Synthetic
atgggtgttagtgatgttccgcgtgatctggaagttgttgcagcaaccccgaccagcctgctgattagctggtcactgccgcatgcaggtcatgcacattattatcgtattacctatggtgaaaccggtggtaatagtccggttcaggaattcaccgttccgggtcgtggtgttaccgcaaccattagcggtctgaaaccgggtgttgattacaccattaccgtttatgcagttaccctgaccaaaagcaaaattattcattatatgccgattagcattaattatcgcaccgaaattgataaaccgagccagcatcatcatcaccatcat

SEQ ID NO: 138 - DNA, 330 bp, Artificial Sequence
  Synthetic
atgggtgttagtgatgttccgcgtgatctggaagttgttgcagcaaccccgaccagcctgctgattagctggtcactgccgtatccgggtcatctgaattattatcgtattacctatggtgaaaccggtggtaatagtccggttcaggaattcaccgttccgggtcgtggtgttaccgcaaccattagcggtctgaaaccgggtgttgattacaccattaccgtttatgcagttaccctgaccaaaagcaaaattattcattatatgccgattagcattaattatcgcaccgaaattgataaaccgagccagcatcatcatcaccatcat

SEQ ID NO: 139 - DNA, 330 bp, Artificial Sequence
  Synthetic
atgggtgttagtgatgttccgcgtgatctggaagttgttgcagcaaccccgaccagcctgctgattagctggaccctgccgcatgcaggtcgtgcacattattatcgtattacctatggtgaaaccggtggtaatagtccggttcaggaattcaccgttccgggtcgtggtgttaccgcaaccattagcggtctgaaaccgggtgttgattacaccattaccgtttatgcagttaccctgacccgcagcaaaattattcattatatgccgattagcattaattatcgcaccgaaattgataaaccgagccagcatcatcatcaccatcat

SEQ ID NO: 140 - DNA, 330 bp, Artificial Sequence
  Synthetic
atgggtgttagtgatgttccgcgtgatctggaagttgttgcagcaaccccgaccagcctgctgattagctggtcactgccgtatgcaggtcatgcacattattatcgtattacctatggtgaaaccggtggtaatagtccggttcaggaattcaccgttccgggtcgtggtgttaccgcaaccattagcggtctgaaaccgggtgttgattacaccattaccgtttatgcagttaccctgaccaaaagcaaaattattcattatatgccgattagcattaattatcgcaccgaaattgataaaccgagccagcatcatcatcaccatcat

SEQ ID NO: 141 - DNA, 330 bp, Artificial Sequence
  Synthetic
atgggtgttagtgatgttccgcgtgatctggaagttgttgcagcaaccccgaccagcctgctgattagctggtcactgccgcatgcaggtcatgcacattattatcgtattacctatggtgaaaccggtggtaatagtccggttcaggaattcaccgttccgggtcgtggtgttaccgcaaccattagcggtctgaaaccgggtgttgattacaccattaccgtttatgcagttaccctgacccgcagcaaaattattcattatatgccgattagcattaattatcgcaccgaaattgataaaccgagccagcatcatcatcaccatcat

SEQ ID NO: 142 - DNA, 330 bp, Artificial Sequence
  Synthetic
atgggtgttagtgatgttccgcgtgatctggaagttgttgcagcaaccccgaccagcctgctgattagctggtcactgccgtatccgggtcatctgaattattatcgtattacctatggtgaaaccggtggtaatagtccggttcaggaattcaccgttccgggtcgtggtgttaccgcaaccattagcggtctgaaaccgggtgttgattacaccattaccgtttatgcagttaccctgacccgcagcaaaattattcattatatgccgattagcattaattatcgcaccgaaattgataaaccgagccagcatcatcatcaccatcat

SEQ ID NO: 143 - DNA, 330 bp, Artificial Sequence
  Synthetic
atgggtgttagtgatgttccgcgtgatctggaagttgttgcagcaaccccgaccagcctgctgattagctggaccctgccgcatgcaggtcgtgcacattattatcgtattacctatggtgaaaccggtggtaatagtccggttcaggaattcaccgttccgggtcgtggtgttaccgcaaccattagcggtctgaaaccgggtgttgattacaccattaccgtttatgcagttaccgttagcagcaccaaagtgattcattataaaccgattagcattaattatcgcaccgaaattgataaaccgagccagcatcatcatcaccatcat

SEQ ID NO: 144 - DNA, 330 bp, Artificial Sequence
  Synthetic
atgggtgttagtgatgttccgcgtgatctggaagttgttgcagcaaccccgaccagcctgctgattagctggtcactgccgtatgcaggtcatgcacattattatcgtattacctatggtgaaaccggtggtaatagtccggttcaggaattcaccgttccgggtcgtggtgttaccgcaaccattagcggtctgaaaccgggtgttgattacaccattaccgtttatgcagttaccctgacccgcagcaaaattattcattatatgccgattagcattaattatcgcaccgaaattgataaaccgagccagcatcatcatcaccatcat

SEQ ID NO: 145 - DNA, 330 bp, Artificial Sequence
  Synthetic
atgggtgttagtgatgttccgcgtgatctggaagttgttgcagcaaccccgaccagcctgctgattagctggtcactgccgcatgcaggtcatgcacattattatcgtattacctatggtgaaaccggtggtaatagtccggttcaggaattcaccgttccgggtcgtggtgttaccgcaaccattagcggtctgaaaccgggtgttgattacaccattaccgtttatgcagttaccctgaccaaaagcaaagtgattcattatatgccgattagcattaattatcgcaccgaaattgataaaccgagccagcatcatcatcaccatcat

SEQ ID NO: 146 - DNA, 330 bp, Artificial Sequence
  Synthetic
atgggtgttagtgatgttccgcgtgatctggaagttgttgcagcaaccccgaccagcctgctgattagctggtcactgccgtatccgggtcatctgaattattatcgtattacctatggtgaaaccggtggtaatagtccggttcaggaattcaccgttccgggtcgtggtgttaccgcaaccattagcggtctgaaaccgggtgttgattacaccattaccgtttatgcagttaccctgaccaaaagcaaagtgattcattatatgccgattagcattaattatcgcaccgaaattgataaaccgagccagcatcatcatcaccatcat

SEQ ID NO: 147 - DNA, 330 bp, Artificial Sequence
  Synthetic
atgggtgttagtgatgttccgcgtgatctggaagttgttgcagcaaccccgaccagcctgctgattagctggaccctgccgcatgcaggtcgtgcacattattatcgtattacctatggtgaaaccggtggtaatagtccggttcaggaattcaccgttccgggtcgtggtgttaccgcaaccattagcggtctgaaaccgggtgttgattacaccattaccgtttatgcagttaccgttagcagcaccaaagttattgtttatctgccgattagcattaattatcgcaccgaaattgataaaccgagccagcatcatcatcaccatcat

SEQ ID NO: 148 - DNA, 330 bp, Artificial Sequence
  Synthetic
atgggtgttagtgatgttccgcgtgatctggaagttgttgcagcaaccccgaccagcctgctgattagctggtcactgccgtatgcaggtcatgcacattattatcgtattacctatggtgaaaccggtggtaatagtccggttcaggaattcaccgttccgggtcgtggtgttaccgcaaccattagcggtctgaaaccgggtgttgattacaccattaccgtttatgcagttaccctgaccaaaagcaaagtgattcattatatgccgattagcattaattatcgcaccgaaattgataaaccgagccagcatcatcatcaccatcat

SEQ ID NO: 149 - DNA, 330 bp, Artificial Sequence
  Synthetic
atgggtgttagtgatgttccgcgtgatctggaagttgttgcagcaaccccgaccagcctgctgattagctggaccctgccgcatgcaggtcgtgcacattattatcgtattacctatggtgaaaccggtggtaatagtccggttcaggaattcaccgttccgggtcgtggtgttaccgcaaccattagcggtctgaaaccgggtgttgattacaccattaccgtttatgcagttaccgttaccaccaccaaagtgattcattataaaccgattagcattaattatcgcaccgaaattgataaaccgagccagcatcatcatcaccatcat

SEQ ID NO: 150 - DNA, 327 bp, Artificial Sequence
  Synthetic
atgggagtttctgatgtgccgcgcgacctggaagtggttgctgccacccccaccagcctgctgatcagctgggacgctccgggtggtctggctcgatattaccgcatcacttacggcgaaacaggaggcaatagccctgtccaggagttcactgtgatcggtcgtggtagcacagctaccatcagcggccttaaacctggcgttgattataccatcactgtgtatgctgtcactatcgaccgtgacggtgtcaaccacttcgccccaatttccattaattaccgcacagaaattgacaaaccatcccagcaccatcaccaccaccac

SEQ ID NO: 151 - DNA, 330 bp, Artificial Sequence
  Synthetic
atgggagtttctgatgtgccgcgcgacctggaagtggttgctgccacccccaccagcctgctgatcagctggtctctgccgactccaggtctcgcccattattaccgcatcacttacggcgaaacaggaggcaatagccctgtccaggagttcactgtgcctggtcgtggtgttacagctaccatcagcggccttaaacctggcgttgattataccatcactgtgtatgctgtcactgtcactcatcacggcgtcatcggctacaaaccaatttccattaattaccgcacagaaattgacaaaccatcccagcaccatcaccaccaccac

SEQ ID NO: 152 - DNA, 330 bp, Artificial Sequence
  Synthetic
atgggagtttctgatgtgccgcgcgacctggaagtggttgctgccacccccaccagcctgctgatcagctggtctctgccgcaccgtggtgtcgccaattattaccgcatcacttacggcgaaacaggaggcaatagccctgtccaggagttcactgtgcctggtcgtggtgttacagctaccatcagcggccttaaacctggcgttgattataccatcactgtgtatgctgtcactctcactggagcgaacgtcatcatctacaaaccaatttccattaattaccgcacagaaattgacaaaccatcccagcaccatcaccaccaccac

SEQ ID NO: 153 - DNA, 330 bp, Artificial Sequence
  Synthetic
atgggagtttctgatgtgccgcgcgacctggaagtggttgctgccacccccaccagcctgctgatcagctggtctctgccgagcagcggtgtcgcccattattaccgcatcacttacggcgaaacaggaggcaatagccctgtccaggagttcactgtgcctggtcgtggtgttacagctaccatcagcggccttaaacctggcgttgattataccatcactgtgtatgctgtcactgtcactaacactggtgtcatcatctacaaaccaatttccattaattaccgcacagaaattgacaaaccatcccagcaccatcaccaccaccac

SEQ ID NO: 154 - DNA, 330 bp, Artificial Sequence
  Synthetic
atgggagtttctgatgtgccgcgcgacctggaagtggttgctgccacccccaccagcctgctgatcagctggtctctgccgcatcacggtttcggccattattaccgcatcacttacggcgaaacaggaggcaatagccctgtccaggagttcactgtgcctggtcgtggtgttacagctaccatcagcggccttaaacctggcgttgattataccatcactgtgtatgctgtcactgtcactgctacggggatcatcatctacaaaccaatttccattaattaccgcacagaaattgacaaaccatcccagcaccatcaccaccaccac

SEQ ID NO: 155 - DNA, 330 bp, Artificial Sequence
  Synthetic
atgggagtttctgatgtgccgcgcgacctggaagtggttgctgccacccccaccagcctgctgatcagctggtctctgccgcacgccggtgacgcccattattaccgcatcacttacggcgaaacaggaggcaatagccctgtccaggagttcactgtgcctggtcgtggtgttacagctaccatcagcggccttaaacctggcgttgattataccatcactgtgtatgctgtcactgttactagagcgggtttctaccgctacaaaccaatttccattaattaccgcacagaaattgacaaaccatcccagcaccatcaccaccaccac

SEQ ID NO: 156 - DNA, 330 bp, Artificial Sequence
  Synthetic
atgggagtttctgatgtgccgcgcgacctggaagtggttgctgccacccccaccagcctgctgatcagctggtctctgccgcataatggtgtcgcccattattaccgcatcacttacggcgaaacaggaggcaatagccctgtccaggagttcactgtgcctggtcgtggtgttacagctaccatcagcggccttaaacctggcgttgattataccatcactgtgtatgctgtcactgtcactcgggaggaagtcatcagctacaaaccaatttccattaattaccgcacagaaattgacaaaccatcccagcaccatcaccaccaccac

SEQ ID NO: 157 - DNA, 330 bp, Artificial Sequence
  Synthetic
atgggagtttctgatgtgccgcgcgacctggaagtggttgctgccacccccaccagcctgctgatcagctggtctctgccgcgtcagggtctcgccaattattaccgcatcacttacggcgaaacaggaggcaatagccctgtccaggagttcactgtgcctggtcgtggtgttacagctaccatcagcggccttaaacctggcgttgattataccatcactgtgtatgctgtcactgtcactgctgctggggtcatcatctacaaaccaatttccattaattaccgcacagaaattgacaaaccatcccagcaccatcaccaccaccac

SEQ ID NO: 158 - DNA, 330 bp, Artificial Sequence
  Synthetic
atgggagtttctgatgtgccgcgcgacctggaagtggttgctgccacccccaccagcctgctgatcagctggtctctgccgggaccgggtcacttccattattaccgcatcacttacggcgaaacaggaggcaatagccctgtccaggagttcactgtgcctggtcgtggtgttacagctaccatcagcggccttaaacctggcgttgattataccatcactgtgtatgctgtcactgtcactgctaaccagcccatcatctacaaaccaatttccattaattaccgcacagaaattgacaaaccatcccagcaccatcaccaccaccac

SEQ ID NO: 159 - DNA, 330 bp, Artificial Sequence
  Synthetic
atgggagtttctgatgtgccgcgcgacctggaagtggttgctgccacccccaccagcctgctgatcagctggtctctgccgcaccccggtctcggccattattaccgcatcacttacggcgaaacaggaggcaatagccctgtccaggagttcactgtgcctggtcgtggtgttacagctaccatcagcggccttaaacctggcgttgattataccatcactgtgtatgctgtcactatcactccggaaacgatcatcgtctacaaaccaatttccattaattaccgcacagaaattgacaaaccatcccagcaccatcaccaccaccac

SEQ ID NO: 160 - DNA, 327 bp, Artificial Sequence
  Synthetic
atgggagtttctgatgtgccgcgcgacctggaagtggttgctgccacccccaccagcctgctgatcagctgggacgctccgagaggtctggctcgatattaccgcatcacttacggcgaaacaggaggcaatagccctgtccaggagttcactgtgttcggtcgtggtaccacagctaccatcagcggccttaaacctggcgttgattataccatcactgtgtatgctgtcactatcgaccgtgacggtacccgcagcttcgacccaatttccattaattaccgcacagaaattgacaaaccatcccagcaccatcaccaccaccac

SEQ ID NO: 161 - DNA, 327 bp, Artificial Sequence
  Synthetic
atgggagtttctgatgtgccgcgcgacctggaagtggttgctgccacccccaccagcctgctgatcagctgggacgctccggctggtctggctcgatattaccgcatcacttacggcgaaacaggaggcaatagccctgtccaggagttcactgtggtcggtcgtggtaacacagctaccatcagcggccttaaacctggcgttgattataccatcactgtgtatgctgtcactatcttccgtgacggtcccgtcacctgggacccaatttccattaattaccgcacagaaattgacaaaccatcccagcaccatcaccaccaccac

SEQ ID NO: 162 - DNA, 330 bp, Artificial Sequence
  Synthetic
atgggagtttctgatgtgccgcgcgacctggaagtggttgctgccacccccaccagcctgctgatcagctggtctctgccgcaccaaggtaaagccaattattaccgcatcacttacggcgaaacaggaggcaatagccctgtccaggagttcactgtgcctggtcgtggtgttacagctaccatcagcggccttaaacctggcgttgattataccatcactgtgtatgctgtcactgttactgatacagggtacctcaagtacaaaccaatttccattaattaccgcacagaaattgacaaaccatcccagcaccatcaccaccaccac

SEQ ID NO: 163 - DNA, 327 bp, Artificial Sequence
  Synthetic
atgggagtttctgatgtgccgcgcgacctggaagtggttgctgccacccccaccagcctgctgatcagctgggacgctccgaagggtctggctcgatattaccgcatcacttacggcgaaacaggaggcaatagccctgtccaggagttcactgtggtcggtcgtggtaacacagctaccatcagcggccttaaacctggcgttgattataccatcactgtgtatgctgtcactatcttccgtgacggtcccgtcacctgggacccaatttccattaattaccgcacagaaattgacaaaccatcccagcaccatcaccaccaccac

SEQ ID NO: 164 - DNA, 330 bp, Artificial Sequence
  Synthetic
atgggagtttctgatgtgccgcgcgacctggaagtggttgctgccacccccaccagcctgctgatcagctggtctctgccgaatcccggtatcgcccattattaccgcatcacttacggcgaaacaggaggcaatagccctgtccaggagttcactgtgcctggtcgtggtgttacagctaccatcagcggccttaaacctggcgttgattataccatcactgtgtatgctgtcactctcactggcagtgacaccatcttctacaaaccaatttccattaattaccgcacagaaattgacaaaccatcccagcaccatcaccaccaccac

SEQ ID NO: 165 - DNA, 330 bp, Artificial Sequence
  Synthetic
atgggagtttctgatgtgccgcgcgacctggaagtggttgctgccacccccaccagcctgctgatcagctggtctctgccgcggccgggtaacgcccattattaccgcatcacttacggcgaaacaggaggcaatagccctgtccaggagttcactgtgcctggtcgtggtgttacagctaccatcagcggccttaaacctggcgttgattataccatcactgtgtatgctgtcactgttactggcaaagatgtcatcaagtacaaaccaatttccattaattaccgcacagaaattgacaaaccatcccagcaccatcaccaccaccac

SEQ ID NO: 166 - DNA, 327 bp, Artificial Sequence
  Synthetic
atgggagtttctgatgtgccgcgcgacctggaagtggttgctgccacccccaccagcctgctgatcagctgggacgctccggctggtctggctcgatattaccgcatcacttacggcgaaacaggaggcaatagccctgtccaggagttcactgtggtcggtcgtggtaacacagctaccatcagcggccttaaacctggcgttgattataccatcactgtgtatgctgtcactatcttccgtgacggtgtcgtcaactacggcccaatttccattaattaccgcacagaaattgacaaaccatcccagcaccatcaccaccaccac

SEQ ID NO: 167 - DNA, 330 bp, Artificial Sequence
  Synthetic
atgggagtttctgatgtgccgcgcgacctggaagtggttgctgccacccccaccagcctgctgatcagctggtctctgccgaatccgggtaacgcccattattaccgcatcacttacggcgaaacaggaggcaatagccctgtccaggagttcactgtgcctggtcgtggtgttacagctaccatcagcggccttaaacctggcgttgattataccatcactgtgtatgctgtcactgttactgacacaggtttcatcacgtacaaaccaatttccattaattaccgcacagaaattgacaaaccatcccagcaccatcaccaccaccac

SEQ ID NO: 168 - protein, 5 aa, Artificial Sequence
  Synthetic
INYRT

SEQ ID NO: 169 - protein, 227 aa, Artificial Sequence
  Synthetic
DKTHTCPPCPAPELLGGPSVFLFPPKPKDTLMISRTPEVTCVVVDVSHEDPEVKFNWYVDGVEVHNAKTKPREEQYNSTYRVVSVLTVLHQDWLNGKEYKCKVSNKALPAPIEKTISKAKGQPREPQVYTLPPSRDELTKNQVSLTCLVKGFYPSDIAVEWESNGQPENNYKTTPPVLDSDGSFFLYSKLTVDKSRWQQGNVFSCSVMHEALHNHYTQKSLSLSPGK

SEQ ID NO: 170 - protein, 16 aa, Artificial Sequence
  Synthetic
DKTHTCPPCPAPELLG

SEQ ID NO: 171 - protein, 24 aa, Artificial Sequence
  Synthetic
EPKSSDKTHTCPPCPAPELLGGPS

SEQ ID NO: 172 - protein, 24 aa, Artificial Sequence
  Synthetic
EPKSSDKTHTCPPCPAPELLGGSS

SEQ ID NO: 173 - protein, 24 aa, Artificial Sequence
  Synthetic
EPKSSGSTHTCPPCPAPELLGGSS

SEQ ID NO: 174 - protein, 19 aa, Artificial Sequence
  Synthetic
DKTHTCPPCPAPELLGGPS

SEQ ID NO: 175 - protein, 19 aa, Artificial Sequence
  Synthetic
DKTHTCPPCPAPELLGGSS

SEQ ID NO: 176 - protein, 330 aa, Artificial Sequence [sequence omitted]

SEQ ID NO: 177 - protein, 20 aa, Artificial Sequence
  Synthetic
METDTLLLWVLLLWVPGSTG

SEQ ID NO: 178 - protein, 208 aa, Artificial Sequence
  Synthetic
VFLFPPKPKDTLMISRTPEVTCVVVDVSHEDPEVKFNWYVDGVEVHNAKTKPREEQYNSTYRVVSVLTVLHQDWLNGKEYKCKVSNKALPAPIEKTISKAKGQPREPQVYTLPPSRDELTKNQVSLTCLVKGFYPSDIAVEWESNGQPENNYKTTPPVLDSDGSFFLYSKLTVDKSRWQQGNVFSCSVMHEALHNHYTQKSLSLSPGK

SEQ ID NO: 179 - protein, 206 aa, Artificial Sequence
  Synthetic
VFLFPPKPKDTLMISRTPEVTCVVVDVSHEDPEVKFNWYVDGVEVHNAKTKPREEQYNSTYRVVSVLTVLHQDWLNGKEYKCKVSNKALPAPIEKTISKAKGQPREPQVYTLPPSRDELTKNQVSLTCLVKGFYPSDIAVEWESNGQPENNYKTTPPVLDSDGSFFLYSKLTVDKSRWQQGNVFSCSVMHEALHNHYTQKSLSLSP

SEQ ID NO: 180 - protein, 16 aa, Artificial Sequence
  Synthetic
GSTHTCPPCPAPELLG

SEQ ID NO: 181 - protein, 8 aa, Artificial Sequence
  Synthetic
GAGGGGSG

SEQ ID NO: 182 - protein, 6 aa, Artificial Sequence
  Synthetic
EPKSSD

SEQ ID NO: 183 - protein, 21 aa, Artificial Sequence
  Synthetic
ESPKAQASSVPTAQPQAEGLA

SEQ ID NO: 184 - protein, 17 aa, Artificial Sequence
  Synthetic
ELQLEESAAEAQDGELD

SEQ ID NO: 185 - protein, 9 aa, Artificial Sequence
  Synthetic
GQPDEPGGS

SEQ ID NO: 186 - protein, 13 aa, Artificial Sequence
  Synthetic
GGSGSGSGSGSGS

SEQ ID NO: 187 - protein, 17 aa, Artificial Sequence
  Synthetic
ELQLEESAAEAQEGELE

SEQ ID NO: 188 - protein, 5 aa, Artificial Sequence
  Synthetic
GSGSG

SEQ ID NO: 189 - protein, 4 aa, Artificial Sequence
  Synthetic
GSGC

SEQ ID NO: 190 - protein, 7 aa, Artificial Sequence
  Synthetic
AGGGGSG

SEQ ID NO: 191 - protein, 4 aa, Artificial Sequence
  Synthetic
GSGS

SEQ ID NO: 192 - protein, 8 aa, Artificial Sequence
  Synthetic
QPDEPGGS

SEQ ID NO: 193 - protein, 6 aa, Artificial Sequence
  Synthetic
GSGSGS

SEQ ID NO: 194 - protein, 6 aa, Artificial Sequence
  Synthetic
TVAAPS

SEQ ID NO: 195 - protein, 8 aa, Artificial Sequence
  Synthetic
KAGGGGSG

SEQ ID NO: 196 - protein, 13 aa, Artificial Sequence
  Synthetic
KGSGSGSGSGSGS

SEQ ID NO: 197 - protein, 9 aa, Artificial Sequence
  Synthetic
KQPDEPGGS

SEQ ID NO: 198 - protein, 18 aa, Artificial Sequence
  Synthetic
KELQLEESAAEAQDGELD

SEQ ID NO: 199 - protein, 7 aa, Artificial Sequence
  Synthetic
KTVAAPS

SEQ ID NO: 200 - protein, 9 aa, Artificial Sequence
  Synthetic
KAGGGGSGG

SEQ ID NO: 201 - protein, 14 aa, Artificial Sequence
  Synthetic
KGSGSGSGSGSGSG

SEQ ID NO: 202 - protein, 10 aa, Artificial Sequence
  Synthetic
KQPDEPGGSG

SEQ ID NO: 203 - protein, 19 aa, Artificial Sequence
  Synthetic
KELQLEESAAEAQDGELDG

SEQ ID NO: 204 - protein, 8 aa, Artificial Sequence
  Synthetic
KTVAAPSG

SEQ ID NO: 205 - protein, 8 aa, Artificial Sequence
  Synthetic
AGGGGSGG

SEQ ID NO: 206 - protein, 7 aa, Artificial Sequence
  Synthetic
AGGGGSG

SEQ ID NO: 207 - protein, 13 aa, Artificial Sequence
  Synthetic
GSGSGSGSGSGSG

SEQ ID NO: 208 - protein, 9 aa, Artificial Sequence
  Synthetic
QPDEPGGSG

SEQ ID NO: 209 - protein, 7 aa, Artificial Sequence
  Synthetic
TVAAPSG

SEQ ID NO: 210 - protein, 7 aa, Artificial Sequence
  Synthetic
PSTSTST

SEQ ID NO: 211 - protein, 7 aa, Artificial Sequence
  Synthetic
EIDKPSQ

SEQ ID NO: 212 - protein, 8 aa, Artificial Sequence
  Synthetic
GSGSGSGS

SEQ ID NO: 213 - protein, 10 aa, Artificial Sequence
  Synthetic
GSGSGSGSGS

SEQ ID NO: 214 - protein, 12 aa, Artificial Sequence
  Synthetic
GSGSGSGSGSGS

SEQ ID NO: 215 - protein, 14 aa, Artificial Sequence
  Synthetic
GSGSGSGSGSGSGS

SEQ ID NO: 216 - protein, 13 aa, Artificial Sequence
  Synthetic
GGSGSGSGSGSGS

SEQ ID NO: 217 - protein, 16 aa, Artificial Sequence
  Synthetic
GGSGSGSGSGSGSGSG

SEQ ID NO: 218 - protein, 15 aa, Artificial Sequence
  Synthetic
GSEGSEGSEGSEGSE

SEQ ID NO: 219 - protein, 8 aa, Artificial Sequence
  Synthetic
GGSEGGSE

SEQ ID NO: 220 - protein, 35 aa, Artificial Sequence
  Synthetic
GGGGSGGGGSGGGGSGGGGSGGGGSGGGGSGGGGS

SEQ ID NO: 221 - protein, 25 aa, Artificial Sequence
  Synthetic
GGGGSGGGGSGGGGSGGGGSGGGGS

SEQ ID NO: 222 - protein, 16 aa, Artificial Sequence
  Synthetic
GGGGSGGGGSGGGGSG

SEQ ID NO: 223 - protein, 7 aa, Artificial Sequence
  Synthetic
GPGPGPG

SEQ ID NO: 224 - protein, 11 aa, Artificial Sequence
  Synthetic
GPGPGPGPGPG

SEQ ID NO: 225 - protein, 6 aa, Artificial Sequence
  Synthetic
PAPAPA

SEQ ID NO: 226 - protein, 12 aa, Artificial Sequence
  Synthetic
PAPAPAPAPAPA

SEQ ID NO: 227 - protein, 18 aa, Artificial Sequence
  Synthetic
PAPAPAPAPAPAPAPAPA

SEQ ID NO: 228 - protein, 106 aa, Artificial Sequence
  Synthetic
MGVSDVPRDLEVVAATPTSLLISWVSPRGRARYYRITYGETGGNSPVQEFTVPGRGSTATISGLKPGVDYTITVYAVTIYRDGMSHHDPISINYRTGSGCHHHHHH

SEQ ID NO: 229 - protein, 107 aa, Artificial Sequence
  Synthetic
MGVSDVPRDLEVVAATPTSLLISWSLPHAGHVNYYRITYGETGGNSPVQEFTVPGRGVTATISGLKPGVDYTITVYAVTLTKSQMIHYMPISINYRTGSGCHHHHHH

SEQ ID NO: 230 - protein, 108 aa, Artificial Sequence
  Synthetic
MGVSDVPRDLEVVAATPTSLLISWTLPHAGRAHYYRITYGETGGNSPVQEFTVPGRGVTATISGLKPGVDYTITVYAVTVTTTSVILYKPISINYRTEGSGCHHHHHH

SEQ ID NO: 231 - protein, 108 aa, Artificial Sequence
  Synthetic
MGVSDVPRDLEVVAATPTSLLISWYLPYPAHMNYYRITYGETGGNSPVQEFTVPGRGLTATISGLKPGVDYTITVYAVTLTKSQILHHRPISINYRTEGSGCHHHHHH

SEQ ID NO: 232 - protein, 108 aa, Artificial Sequence
  Synthetic
MGVSDVPRDLEVVAATPTSLLISWSLPYAGHLNYYRITYGETGGNSPVQEFTVPGRGVTATISGLKPGVDYTITVYAVTLTKSQLIHYMPISINYRTEGSGCHHHHHH

SEQ ID NO: 233 - protein, 108 aa, Artificial Sequence
  Synthetic
MGVSDVPRDLEVVAATPTSLLISWTLPHAGRAHYYRITYGETGGNSPVQEFTVPGRGVTATISGLKPGVDYTITVYAVTVTTTKVIHYKPISINYRTEGSGCHHHHHH

SEQ ID NO: 234 - protein, 108 aa, Artificial Sequence; identical to SEQ ID NO: 233
  Synthetic

SEQ ID NO: 235 - protein, 107 aa, Artificial Sequence
  Synthetic
MGVSDVPRDLEVVAATPTSLLISWDAPRGLARYYRITYGETGGNSPVQEFTVFGRGTTATISGLKPGVDYTITVYAVTIDRDGTRSFDPISINYRTEGSGCHHHHHH

SEQ ID NO: 236 - protein, 107 aa, Artificial Sequence
  Synthetic
MGVSDVPRDLEVVAATPTSLLISWDAPAGLARYYRITYGETGGNSPVQEFTVVGRGNTATISGLKPGVDYTITVYAVTIFRDGPVTWDPISINYRTEGSGCHHHHHH

SEQ ID NO: 237 - protein, 107 aa, Artificial Sequence
  Synthetic
MGVSDVPRDLEVVAATPTSLLISWDAPKGLARYYRITYGETGGNSPVQEFTVVGRGNTATISGLKPGVDYTITVYAVTIFRDGPVTWDPISINYRTEGSGCHHHHHH

SEQ ID NO: 238 - protein, 108 aa, Artificial Sequence
  Synthetic
MGVSDVPRDLEVVAATPTSLLISWSLPNPGNAHYYRITYGETGGNSPVQEFTVPGRGVTATISGLKPGVDYTITVYAVTVTDTGFITYKPISINYRTEGSGCHHHHHH

SEQ ID NO: 239 - protein, 108 aa, Artificial Sequence
  Synthetic
MGVSDVPRDLEVVAATPTSLLISWSLPHQGKANYYRITYGETGGNSPVQEFTVPGRGVTATISGLKPGVDYTITVYAVTVTDTGYLKYKPISINYRTEGSGCHHHHHH

SEQ ID NO: 240 - DNA, 318 bp, Artificial Sequence
  Synthetic
atgggagtttctgatgtgccgcgcgacctggaagtggttgctgccacccccaccagcctgctgatcagctgggtttctccgcgtggtcgtgctcgatattaccgcatcacttacggcgaaacaggaggcaatagccctgtccaggagttcactgtgcctggtcgtggttctacagctaccatcagcggccttaaacctggcgttgattataccatcactgtgtatgctgtcactatctaccgtgacggtatgtctcatcatgacccaatttccattaattaccgcacaggtagcggttgccaccatcaccaccatcac

SEQ ID NO: 241 - DNA, 321 bp, Artificial Sequence
  Synthetic
atgggagtttctgatgtgccgcgcgacctggaagtggttgctgccacccccaccagcctgctgatcagctggtctctgccgcatgctggtcatgtgaactattaccgcatcacttacggcgaaacaggaggcaatagccctgtccaggagttcactgtgcctggtcgtggtgttacagctaccatcagcggccttaaacctggcgttgattataccatcactgtgtatgctgtcactctgactaaatctcagatgatccattacatgccaatttccattaattaccgcacaggtagcggttgccaccatcaccaccatcac

SEQ ID NO: 242 - DNA, 324 bp, Artificial Sequence
  Synthetic
atgggagtttctgatgtgccgcgcgacctggaagtggttgctgccacccccaccagcctgctgatcagctggactttgccgcatgctggtcgtgcgcactattaccgcatcacttacggcgaaacaggaggcaatagccctgtccaggagttcactgtgcctgggcggggtgttacagctaccatcagcggccttaaacctggcgttgattataccatcactgtgtatgctgtcactgtgacgacaacttcggtgatcctttacaagccaatttccattaattaccgcacagaaggtagcggttgccaccatcaccaccatcac

SEQ ID NO: 243 - DNA, 324 bp, Artificial Sequence
  Synthetic
atgggagtttctgatgtgccgcgcgacctggaagtggttgctgccacccccaccagcctgctgatcagctggtacctcccgtatcctgcgcatatgaactattaccgcatcacttacggcgaaacaggaggcaatagccctgtccaggagttcactgtgcctgggcggggtctgacagctaccatcagcggccttaaacctggcgttgattataccatcactgtgtatgctgtcactctgacaaaatctcagattctccatcataggccaatttccattaattaccgcacagaaggtagcggttgccaccatcaccaccatcac

SEQ ID NO: 244 - DNA, 324 bp, Artificial Sequence
  Synthetic
atgggagtttctgatgtgccgcgcgacctggaagtggttgctgccacccccaccagcctgctgatcagctggtctcttccttatgctggtcatctaaactattaccgcatcacttacggcgaaacaggaggcaatagccctgtccaggagttcactgtgcctggtcgtggtgtgacagctaccatcagcggccttaaacctggcgttgattataccatcactgtgtatgctgtcactctgactaagtctcagctgatacattacatgccaatttccattaattaccgcacagaaggtagcggttgccaccatcaccaccatcac

SEQ ID NO: 245 - DNA, 324 bp, Artificial Sequence
  Synthetic
atgggtgttagtgatgttccgcgtgatctggaagttgttgcagcaaccccgaccagcctgctgattagctggaccctgccgcatgcaggtcgtgcacattattatcgtattacctatggtgaaaccggtggtaatagtccggttcaggaattcaccgttccgggtcgtggtgttaccgcaaccattagcggtctgaaaccgggtgttgattacaccattaccgtttatgcagttaccgttaccaccaccaaagtgattcattataaaccgatttccattaattaccgcacagaaggtagcggttgccaccatcaccaccatcac

SEQ ID NO: 246 - DNA, 306 bp, Artificial Sequence
  Synthetic
atgggtgttagtgatgttccgcgtgatctggaagttgttgcagcaaccccgaccagcctgctgattagctggaccctgccgcatgcaggtcgtgcacattattatcgtattacctatggtgaaaccggtggtaatagtccggttcaggaattcaccgttccgggtcgtggtgttaccgcaaccattagcggtctgaaaccgggtgttgattacaccattaccgtttatgcagttaccgttaccaccaccaaagtgattcattataaaccgatttccattaattaccgaacagaaggtagcggttgc

SEQ ID NO: 247 - DNA, 321 bp, Artificial Sequence
  Synthetic
atgggagtttctgatgtgccgcgcgacctggaagtggttgctgccacccccaccagcctgctgatcagctgggacgctccgagaggtctggctcgatattaccgcatcacttacggcgaaacaggaggcaatagccctgtccaggagttcactgtgttcggtcgtggtaccacagctaccatcagcggccttaaacctggcgttgattataccatcactgtgtatgctgtcactatcgaccgtgacggtacccgcagcttcgacccaatttccattaattaccgcacagaaggtagcggttgccaccatcaccaccatcac

SEQ ID NO: 248 - DNA, 321 bp, Artificial Sequence
  Synthetic
atgggagtttctgatgtgccgcgcgacctggaagtggttgctgccacccccaccagcctgctgatcagctgggacgctccggctggtctggctcgatattaccgcatcacttacggcgaaacaggaggcaatagccctgtccaggagttcactgtggtcggtcgtggtaacacagctaccatcagcggccttaaacctggcgttgattataccatcactgtgtatgctgtcactatcttccgtgacggtcccgtcacctgggacccaatttccattaattaccgcacagaaggtagcggttgccaccatcaccaccatcac

SEQ ID NO: 249 - DNA, 321 bp, Artificial Sequence
  Synthetic
atgggagtttctgatgtgccgcgcgacctggaagtggttgctgccacccccaccagcctgctgatcagctgggacgctccgaagggtctggctcgatattaccgcatcacttacggcgaaacaggaggcaatagccctgtccaggagttcactgtggtcggtcgtggtaacacagctaccatcagcggccttaaacctggcgttgattataccatcactgtgtatgctgtcactatcttccgtgacggtcccgtcacctgggacccaatttccattaattaccgcacagaaggtagcggttgccaccatcaccaccatcac

SEQ ID NO: 250 - DNA, 324 bp, Artificial Sequence
  Synthetic
atgggagtttctgatgtgccgcgcgacctggaagtggttgctgccacccccaccagcctgctgatcagctggtctctgccgaatccgggtaacgcccattattaccgcatcacttacggcgaaacaggaggcaatagccctgtccaggagttcactgtgcctggtcgtggtgttacagctaccatcagcggccttaaacctggcgttgattataccatcactgtgtatgctgtcactgttactgacacaggtttcatcacgtacaaaccaatttccattaattaccgcacagaaggtagcggttgccaccatcaccaccatcac

SEQ ID NO: 251 - DNA, 324 bp, Artificial Sequence
  Synthetic
atgggagtttctgatgtgccgcgcgacctggaagtggttgctgccacccccaccagcctgctgatcagctggtctctgccgcaccaaggtaaagccaattattaccgcatcacttacggcgaaacaggaggcaatagccctgtccaggagttcactgtgcctggtcgtggtgttacagctaccatcagcggccttaaacctggcgttgattataccatcactgtgtatgctgtcactgttactgatacagggtacctcaagtacaaaccaatttccattaattaccgcacagaaggtagcggttgccaccatcaccaccatcac

SEQ ID NO: 252 - protein, 336 aa, Artificial Sequence
  Synthetic
EPKSSGSTHTCPPCPAPELLGGSSVFLFPPKPKDTLMISRTPEVTCVVVDVSHEDPEVKFNWYVDGVEVHNAKTKPREEQYNSTYRVVSVLTVLHQDWLNGKEYKCKVSNKALPAPIEKTISKAKGQPREPQVYTLPPSRDELTKNQVSLTCLVKGFYPSDIAVEWESNGQPENNYKTTPPVLDSDGSFFLYSKLTVDKSRWQQGNVFSCSVMHEALHNHYTQKSLSLSPGAGGGGSGGVSDVPRDLEVVAATPTSLLISWSLPYAGHLNYYRITYGETGGNSPVQEFTVPGRGVTATISGLKPGVDYTITVYAVTLTKSQLIHYMPISINYRTEI

SEQ ID NO: 253 - protein, 330 aa, Artificial Sequence
  Synthetic
GVSDVPRDLEVVAATPTSLLISWTLPHAGRAHYYRITYGETGGNSPVQEFTVPGRGVTATISGLKPGVDYTITVYAVTVTTTKVIHYKPISINYRTEIEPKSSDKTHTCPPCPAPELLGGPSVFLFPPKPKDTLMISRTPEVTCVVVDVSHEDPEVKFNWYVDGVEVHNAKTKPREEQYNSTYRVVSVLTVLHQDWLNGKEYKCKVSNKALPAPIEKTISKAKGQPREPQVYTLPPSRDELTKNQVSLTCLVKGFYPSDIAVEWESNGQPENNYKTTPPVLDSDGSFFLYSKLTVDKSRWQQGNVFSCSVMHEALHNHYTQKSLSLSPGK

SEQ ID NO: 254 - protein, 325 aa, Artificial Sequence
  Synthetic
GVSDVPRDLEVVAATPTSLLISWTLPHAGRAHYYRITYGETGGNSPVQEFTVPGRGVTATISGLKPGVDYTITVYAVTVTTTKVIHYKPISINYRTEIDKTHTCPPCPAPELLGGPSVFLFPPKPKDTLMISRTPEVTCVVVDVSHEDPEVKFNWYVDGVEVHNAKTKPREEQYNSTYRVVSVLTVLHQDWLNGKEYKCKVSNKALPAPIEKTISKAKGQPREPQVYTLPPSRDELTKNQVSLTCLVKGFYPSDIAVEWESNGQPENNYKTTPPVLDSDGSFFLYSKLTVDKSRWQQGNVFSCSVMHEALHNHYTQKSLSLSPGK

SEQ ID NO: 255 - protein, 345 aa, Artificial Sequence
  Synthetic
GVSDVPRDLEVVAATPTSLLISWTLPHAGRAHYYRITYGETGGNSPVQEFTVPGRGVTATISGLKPGVDYTITVYAVTVTTTKVIHYKPISINYRTEIESPKAQASSVPTAQPQAEGLAKTHTCPPCPAPELLGGPSVFLFPPKPKDTLMISRTPEVTCVVVDVSHEDPEVKFNWYVDGVEVHNAKTKPREEQYNSTYRVVSVLTVLHQDWLNGKEYKCKVSNKALPAPIEKTISKAKGQPREPQVYTLPPSRDELTKNQVSLTCLVKGFYPSDIAVEWESNGQPENNYKTTPPVLDSDGSFFLYSKLTVDKSRWQQGNVFSCSVMHEALHNHYTQKSLSLSPGK

SEQ ID NO: 256 - protein, 331 aa, Artificial Sequence
  Synthetic
DKTHTCPPCPAPELLGGPSVFLFPPKPKDTLMISRTPEVTCVVVDVSHEDPEVKFNWYVDGVEVHNAKTKPREEQYNSTYRVVSVLTVLHQDWLNGKEYKCKVSNKALPAPIEKTISKAKGQPREPQVYTLPPSRDELTKNQVSLTCLVKGFYPSDIAVEWESNGQPENNYKTTPPVLDSDGSFFLYSKLTVDKSRWQQGNVFSCSVMHEALHNHYTQKSLSLSPGAGGGGSGGVSDVPRDLEVVAATPTSLLISWTLPHAGRAHYYRITYGETGGNSPVQEFTVPGRGVTATISGLKPGVDYTITVYAVTVTTTKVIHYKPISINYRTEI

SEQ ID NO: 257 - protein, 340 aa, Artificial Sequence
  Synthetic
DKTHTCPPCPAPELLGGPSVFLFPPKPKDTLMISRTPEVTCVVVDVSHEDPEVKFNWYVDGVEVHNAKTKPREEQYNSTYRVVSVLTVLHQDWLNGKEYKCKVSNKALPAPIEKTISKAKGQPREPQVYTLPPSRDELTKNQVSLTCLVKGFYPSDIAVEWESNGQPENNYKTTPPVLDSDGSFFLYSKLTVDKSRWQQGNVFSCSVMHEALHNHYTQKSLSLSPELQLEESAAEAQDGELDGVSDVPRDLEVVAATPTSLLISWTLPHAGRAHYYRITYGETGGNSPVQEFTVPGRGVTATISGLKPGVDYTITVYAVTVTTTKVIHYKPISINYRTEI

SEQ ID NO: 258 - protein, 332 aa, Artificial Sequence
  Synthetic
DKTHTCPPCPAPELLGGPSVFLFPPKPKDTLMISRTPEVTCVVVDVSHEDPEVKFNWYVDGVEVHNAKTKPREEQYNSTYRVVSVLTVLHQDWLNGKEYKCKVSNKALPAPIEKTISKAKGQPREPQVYTLPPSRDELTKNQVSLTCLVKGFYPSDIAVEWESNGQPENNYKTTPPVLDSDGSFFLYSKLTVDKSRWQQGNVFSCSVMHEALHNHYTQKSLSLSPGQPDEPGGSGVSDVPRDLEVVAATPTSLLISWTLPHAGRAHYYRITYGETGGNSPVQEFTVPGRGVTATISGLKPGVDYTITVYAVTVTTTKVIHYKPISINYRTEI

SEQ ID NO: 259 - protein, 336 aa, Artificial Sequence
  Synthetic
DKTHTCPPCPAPELLGGPSVFLFPPKPKDTLMISRTPEVTCVVVDVSHEDPEVKFNWYVDGVEVHNAKTKPREEQYNSTYRVVSVLTVLHQDWLNGKEYKCKVSNKALPAPIEKTISKAKGQPREPQVYTLPPSRDELTKNQVSLTCLVKGFYPSDIAVEWESNGQPENNYKTTPPVLDSDGSFFLYSKLTVDKSRWQQGNVFSCSVMHEALHNHYTQKSLSLSPGGSGSGSGSGSGSGVSDVPRDLEVVAATPTSLLISWTLPHAGRAHYYRITYGETGGNSPVQEFTVPGRGVTATISGLKPGVDYTITVYAVTVTTTKVIHYKPISINYRTEI

SEQ ID NO: 260 - protein, 339 aa, Artificial Sequence
  Synthetic
DKTHTCPPCPAPELLGGPSVFLFPPKPKDTLMISRTPEVTCVVVDVSHEDPEVKFNWYVDGVEVHNAKTKPREEQYNSTYRVVSVLTVLHQDWLNGKEYKCKVSNKALPAPIEKTISKAKGQPREPQVYTLPPSRDELTKNQVSLTCLVKGFYPSDIAVEWESNGQPENNYKTTPPVLDSDGSFFLYSKLTVDKSRWQQGNVFSCSVMHEALHNHYTQKSLSLSPELQLEESAAEAQDGELDGVSDVPRDLEVVAATPTSLLISWDAPRGLARYYRITYGETGGNSPVQEFTVFGRGTTATISGLKPGVDYTITVYAVTIDRDGTRSFDPISINYRTEI

SEQ ID NO: 261 - protein, 339 aa, Artificial Sequence
  Synthetic
DKTHTCPPCPAPELLGGPSVFLFPPKPKDTLMISRTPEVTCVVVDVSHEDPEVKFNWYVDGVEVHNAKTKPREEQYNSTYRVVSVLTVLHQDWLNGKEYKCKVSNKALPAPIEKTISKAKGQPREPQVYTLPPSRDELTKNQVSLTCLVKGFYPSDIAVEWESNGQPENNYKTTPPVLDSDGSFFLYSKLTVDKSRWQQGNVFSCSVMHEALHNHYTQKSLSLSPELQLEESAAEAQDGELDGVSDVPRDLEVVAATPTSLLISWDAPAGLARYYRITYGETGGNSPVQEFTVVGRGNTATISGLKPGVDYTITVYAVTIFRDGPVTWDPISINYRTEI

SEQ ID NO: 262 - protein, 339 aa, Artificial Sequence
  Synthetic
DKTHTCPPCPAPELLGGPSVFLFPPKPKDTLMISRTPEVTCVVVDVSHEDPEVKFNWYVDGVEVHNAKTKPREEQYNSTYRVVSVLTVLHQDWLNGKEYKCKVSNKALPAPIEKTISKAKGQPREPQVYTLPPSRDELTKNQVSLTCLVKGFYPSDIAVEWESNGQPENNYKTTPPVLDSDGSFFLYSKLTVDKSRWQQGNVFSCSVMHEALHNHYTQKSLSLSPELQLEESAAEAQDGELDGVSDVPRDLEVVAATPTSLLISWDAPKGLARYYRITYGETGGNSPVQEFTVVGRGNTATISGLKPGVDYTITVYAVTIFRDGPVTWDPISINYRTEI

SEQ ID NO: 263 - protein, 340 aa, Artificial Sequence
  Synthetic
DKTHTCPPCPAPELLGGPSVFLFPPKPKDTLMISRTPEVTCVVVDVSHEDPEVKFNWYVDGVEVHNAKTKPREEQYNSTYRVVSVLTVLHQDWLNGKEYKCKVSNKALPAPIEKTISKAKGQPREPQVYTLPPSRDELTKNQVSLTCLVKGFYPSDIAVEWESNGQPENNYKTTPPVLDSDGSFFLYSKLTVDKSRWQQGNVFSCSVMHEALHNHYTQKSLSLSPELQLEESAAEAQDGELDGVSDVPRDLEVVAATPTSLLISWSLPNPGNAHYYRITYGETGGNSPVQEFTVPGRGVTATISGLKPGVDYTITVYAVTVTDTGFITYKPISINYRTEI

SEQ ID NO: 264 - protein, 340 aa, Artificial Sequence
  Synthetic
DKTHTCPPCPAPELLGGPSVFLFPPKPKDTLMISRTPEVTCVVVDVSHEDPEVKFNWYVDGVEVHNAKTKPREEQYNSTYRVVSVLTVLHQDWLNGKEYKCKVSNKALPAPIEKTISKAKGQPREPQVYTLPPSRDELTKNQVSLTCLVKGFYPSDIAVEWESNGQPENNYKTTPPVLDSDGSFFLYSKLTVDKSRWQQGNVFSCSVMHEALHNHYTQKSLSLSPELQLEESAAEAQDGELDGVSDVPRDLEVVAATPTSLLISWSLPHQGKANYYRITYGETGGNSPVQEFTVPGRGVTATISGLKPGVDYTITVYAVTVTDTGYLKYKPISINYRTEI

SEQ ID NO: 265 - protein, 329 aa, Artificial Sequence
  Synthetic
GVSDVPRDLEVVAATPTSLLISWDAPRGLARYYRITYGETGGNSPVQEFTVFGRGTTATISGLKPGVDYTITVYAVTIDRDGTRSFDPISINYRTEIEPKSSDKTHTCPPCPAPELLGGPSVFLFPPKPKDTLMISRTPEVTCVVVDVSHEDPEVKFNWYVDGVEVHNAKTKPREEQYNSTYRVVSVLTVLHQDWLNGKEYKCKVSNKALPAPIEKTISKAKGQPREPQVYTLPPSRDELTKNQVSLTCLVKGFYPSDIAVEWESNGQPENNYKTTPPVLDSDGSFFLYSKLTVDKSRWQQGNVFSCSVMHEALHNHYTQKSLSLSPGK

SEQ ID NO: 266 - protein, 329 aa, Artificial Sequence
  Synthetic
GVSDVPRDLEVVAATPTSLLISWDAPAGLARYYRITYGETGGNSPVQEFTVVGRGNTATISGLKPGVDYTITVYAVTIFRDGPVTWDPISINYRTEIEPKSSDKTHTCPPCPAPELLGGPSVFLFPPKPKDTLMISRTPEVTCVVVDVSHEDPEVKFNWYVDGVEVHNAKTKPREEQYNSTYRVVSVLTVLHQDWLNGKEYKCKVSNKALPAPIEKTISKAKGQPREPQVYTLPPSRDELTKNQVSLTCLVKGFYPSDIAVEWESNGQPENNYKTTPPVLDSDGSFFLYSKLTVDKSRWQQGNVFSCSVMHEALHNHYTQKSLSLSPGK

SEQ ID NO: 267 - protein, 329 aa, Artificial Sequence
  Synthetic
GVSDVPRDLEVVAATPTSLLISWDAPKGLARYYRITYGETGGNSPVQEFTVVGRGNTATISGLKPGVDYTITVYAVTIFRDGPVTWDPISINYRTEIEPKSSDKTHTCPPCPAPELLGGPSVFLFPPKPKDTLMISRTPEVTCVVVDVSHEDPEVKFNWYVDGVEVHNAKTKPREEQYNSTYRVVSVLTVLHQDWLNGKEYKCKVSNKALPAPIEKTISKAKGQPREPQVYTLPPSRDELTKNQVSLTCLVKGFYPSDIAVEWESNGQPENNYKTTPPVLDSDGSFFLYSKLTVDKSRWQQGNVFSCSVMHEALHNHYTQKSLSLSPGK

SEQ ID NO: 268 - protein, 330 aa, Artificial Sequence
  Synthetic
GVSDVPRDLEVVAATPTSLLISWSLPNPGNAHYYRITYGETGGNSPVQEFTVPGRGVTATISGLKPGVDYTITVYAVTVTDTGFITYKPISINYRTEIEPKSSDKTHTCPPCPAPELLGGPSVFLFPPKPKDTLMISRTPEVTCVVVDVSHEDPEVKFNWYVDGVEVHNAKTKPREEQYNSTYRVVSVLTVLHQDWLNGKEYKCKVSNKALPAPIEKTISKAKGQPREPQVYTLPPSRDELTKNQVSLTCLVKGFYPSDIAVEWESNGQPENNYKTTPPVLDSDGSFFLYSKLTVDKSRWQQGNVFSCSVMHEALHNHYTQKSLSLSPGK

SEQ ID NO: 269 - protein, 330 aa, Artificial Sequence
  Synthetic
GVSDVPRDLEVVAATPTSLLISWSLPHQGKANYYRITYGETGGNSPVQEFTVPGRGVTATISGLKPGVDYTITVYAVTVTDTGYLKYKPISINYRTEIEPKSSDKTHTCPPCPAPELLGGPSVFLFPPKPKDTLMISRTPEVTCVVVDVSHEDPEVKFNWYVDGVEVHNAKTKPREEQYNSTYRVVSVLTVLHQDWLNGKEYKCKVSNKALPAPIEKTISKAKGQPREPQVYTLPPSRDELTKNQVSLTCLVKGFYPSDIAVEWESNGQPENNYKTTPPVLDSDGSFFLYSKLTVDKSRWQQGNVFSCSVMHEALHNHYTQKSLSLSPGK

SEQ ID NO: 270 - protein, 340 aa, Artificial Sequence
  Synthetic
DKTHTCPPCPAPELLGGPSVFLFPPKPKDTLMISRTPEVTCVVVDVSHEDPEVKFNWYVDGVEVHNAKTKPREEQYNSTYRVVSVLTVLHQDWLNGKEYKCKVSNKALPAPIEKTISKAKGQPREPQVYTLPPSRDELTKNQVSLTCLVKGFYPSDIAVEWESNGQPENNYKTTPPVLDSDGSFFLYSKLTVDKSRWQQGNVFSCSVMHEALHNHYTQKSLSLSPELQLEESAAEAQEGELEGVSDVPRDLEVVAATPTSLLISWTLPHAGRAHYYRITYGETGGNSPVQEFTVPGRGVTATISGLKPGVDYTITVYAVTVTTTKVIHYKPISINYRTEI

SEQ ID NO: 271 - protein, 339 aa, Artificial Sequence
  Synthetic
DKTHTCPPCPAPELLGGPSVFLFPPKPKDTLMISRTPEVTCVVVDVSHEDPEVKFNWYVDGVEVHNAKTKPREEQYNSTYRVVSVLTVLHQDWLNGKEYKCKVSNKALPAPIEKTISKAKGQPREPQVYTLPPSRDELTKNQVSLTCLVKGFYPSDIAVEWESNGQPENNYKTTPPVLDSDGSFFLYSKLTVDKSRWQQGNVFSCSVMHEALHNHYTQKSLSLSPELQLEESAAEAQEGELEGVSDVPRDLEVVAATPTSLLISWDAPAGLARYYRITYGETGGNSPVQEFTVVGRGNTATISGLKPGVDYTITVYAVTIFRDGPVTWDPISINYRTEI

SEQ ID NO: 272 - protein, 339 aa, Artificial Sequence
  Synthetic
DKTHTCPPCPAPELLGGPSVFLFPPKPKDTLMISRTPEVTCVVVDVSHEDPEVKFNWYVDGVEVHNAKTKPREEQYNSTYRVVSVLTVLHQDWLNGKEYKCKVSNKALPAPIEKTISKAKGQPREPQVYTLPPSRDELTKNQVSLTCLVKGFYPSDIAVEWESNGQPENNYKTTPPVLDSDGSFFLYSKLTVDKSRWQQGNVFSCSVMHEALHNHYTQKSLSLSPELQLEESAAEAQEGELEGVSDVPRDLEVVAATPTSLLISWDAPKGLARYYRITYGETGGNSPVQEFTVVGRGNTATISGLKPGVDYTITVYAVTIFRDGPVTWDPISINYRTEI

SEQ ID NO: 273 - protein, 340 aa, Artificial Sequence
  Synthetic
DKTHTCPPCPAPELLGGPSVFLFPPKPKDTLMISRTPEVTCVVVDVSHEDPEVKFNWYVDGVEVHNAKTKPREEQYNSTYRVVSVLTVLHQDWLNGKEYKCKVSNKALPAPIEKTISKAKGQPREPQVYTLPPSRDELTKNQVSLTCLVKGFYPSDIAVEWESNGQPENNYKTTPPVLDSDGSFFLYSKLTVDKSRWQQGNVFSCSVMHEALHNHYTQKSLSLSPELQLEESAAEAQEGELEGVSDVPRDLEVVAATPTSLLISWSLPHQGKANYYRITYGETGGNSPVQEFTVPGRGVTATISGLKPGVDYTITVYAVTVTDTGYLKYKPISINYRTEI

SEQ ID NO: 274 - protein, 230 aa, Artificial Sequence
  Synthetic
EPKSSGSTHTCPPCPAPELLGGSSVFLFPPKPKDTLMISRTPEVTCVVVDVSHEDPEVKFNWYVDGVEVHNAKTKPREEQYNSTYRVVSVLTVLHQDWLNGKEYKCKVSNKALPAPIEKTISKAKGQPREPQVYTLPPSRDELTKNQVSLTCLVKGFYPSDIAVEWESNGQPENNYKTTPPVLDSDGSFFLYSKLTVDKSRWQQGNVFSCSVMHEALHNHYTQKSLSLSP

SEQ ID NO: 275 - protein, 98 aa, Artificial Sequence
  Synthetic
GVSDVPRDLEVVAATPTSLLISWTLPHAGRAHYYRITYGETGGNSPVQEFTVPGRGVTATISGLKPGVDYTITVYAVTVTTTKVIHYKPISINYRTEI

SEQ ID NO: 276 - protein, 225 aa, Artificial Sequence
  Synthetic
DKTHTCPPCPAPELLGGPSVFLFPPKPKDTLMISRTPEVTCVVVDVSHEDPEVKFNWYVDGVEVHNAKTKPREEQYNSTYRVVSVLTVLHQDWLNGKEYKCKVSNKALPAPIEKTISKAKGQPREPQVYTLPPSRDELTKNQVSLTCLVKGFYPSDIAVEWESNGQPENNYKTTPPVLDSDGSFFLYSKLTVDKSRWQQGNVFSCSVMHEALHNHYTQKSLSLSP

SEQ ID NO: 277 - protein, 97 aa, Artificial Sequence
  Synthetic
GVSDVPRDLEVVAATPTSLLISWDAPRGLARYYRITYGETGGNSPVQEFTVFGRGTTATISGLKPGVDYTITVYAVTIDRDGTRSFDPISINYRTEI

SEQ ID NO: 278 - protein, 97 aa, Artificial Sequence
  Synthetic
GVSDVPRDLEVVAATPTSLLISWDAPAGLARYYRITYGETGGNSPVQEFTVVGRGNTATISGLKPGVDYTITVYAVTIFRDGPVTWDPISINYRTEI

SEQ ID NO: 279 - protein, 97 aa, Artificial Sequence
  Synthetic
GVSDVPRDLEVVAATPTSLLISWDAPKGLARYYRITYGETGGNSPVQEFTVVGRGNTATISGLKPGVDYTITVYAVTIFRDGPVTWDPISINYRTEI

SEQ ID NO: 280 - protein, 98 aa, Artificial Sequence
  Synthetic
GVSDVPRDLEVVAATPTSLLISWSLPNPGNAHYYRITYGETGGNSPVQEFTVPGRGVTATISGLKPGVDYTITVYAVTVTDTGFITYKPISINYRTEI

SEQ ID NO: 281 - protein, 98 aa, Artificial Sequence
  Synthetic
GVSDVPRDLEVVAATPTSLLISWSLPHQGKANYYRITYGETGGNSPVQEFTVPGRGVTATISGLKPGVDYTITVYAVTVTDTGYLKYKPISINYRTEI

SEQ ID NO: 282 - protein, 98 aa, Artificial Sequence
  Synthetic
GVSDVPRDLEVVAATPTSLLISWSLPYAGHLNYYRITYGETGGNSPVQEFTVPGRGVTATISGLKPGVDYTITVYAVTLTKSQLIHYMPISINYRTEI

SEQ ID NO: 283 - protein, 226 aa, Artificial Sequence [sequence omitted]

SEQ ID NO: 284 - DNA, 1008 bp, Artificial Sequence
  Synthetic
gagcccaaatctagcgggtcgactcacacatgcccaccgtgcccagcacctgaactcctggggggaagctcagtcttcctcttccccccaaaacccaaggacaccctcatgatctcccggacccctgaggtcacatgcgtggtggtggacgtgagccacgaagaccctgaggtcaagttcaactggtacgtggacggcgtggaggtgcataatgccaagacaaagccgcgggaggagcagtacaacagcacgtaccgtgtggtcagcgtcctcaccgtcctgcaccaggactggctgaatggcaaggagtacaagtgcaaggtctccaacaaagccctcccagcccccatcgagaaaaccatctccaaagccaaagggcagccccgagaaccacaggtgtacaccctgcccccatcccgggatgagctgaccaagaaccaggtcagcctgacctgcctggtcaaaggcttctatcccagcgacatcgccgtggagtgggagagcaatgggcagccggagaacaactacaagaccacgcctcccgtgctggactccgacggctccttcttcctctacagcaagctcaccgtggacaagagcaggtggcagcaggggaacgtcttctcatgctccgtgatgcatgaggctctgcacaaccactacacgcagaagagcctctccctgtctcccggcgccggaggcggcggatccggtggagtttctgatgtgccgcgcgacctggaagtggttgctgccacccccaccagcctgctgatcagctggtctcttccttatgctggtcatctaaactattaccgcatcacttacggcgaaacaggaggcaatagccctgtccaggagttcactgtgcctggtcgtggtgtgacagctaccatcagcggccttaaacctggcgttgattataccatcactgtgtatgctgtcactctgactaagtctcagctgatacattacatgccaatttccattaattaccggaccgaaatc

SEQ ID NO: 285 - DNA, 990 bp, Artificial Sequence
  Synthetic
ggcgtgagcgacgtgccccgggatctagaagtggtggctgctacccccacaagcttgctgatctcctggacactgcctcacgctggccgggctcattactatagaattacctacggggagacaggcgggaactctcccgtgcaggaattcaccgtgcctggaaggggcgtgactgccaccatcagtgggctgaagccaggagtggactacacaattaccgtgtacgctgtgactgtgaccacaactaaagtgatccactacaaacccatctctattaattatcggaccgaaattgagcctaagagctccgacaaaacccacacatgcccaccttgtccagcccccgaactgctgggcggcccttcagtcttcctcttccccccaaaacccaaggacaccctcatgatctcccggacccctgaggtcacatgcgtggtggtggacgtgagccacgaagaccctgaggtcaagttcaactggtacgtggacggcgtggaggtgcataatgccaagacaaagccgcgggaggagcagtacaacagcacgtaccgtgtggtcagcgtcctcaccgtcctgcaccaggactggctgaatggcaaggagtacaagtgcaaggtctccaacaaagccctcccagcccccatcgagaaaaccatctccaaagccaaagggcagccccgagaaccacaggtgtacaccctgcccccatcccgggatgagctgaccaagaaccaggtcagcctgacctgcctggtcaaaggcttctatcccagcgacatcgccgtggagtgggagagcaatgggcagccggagaacaactacaagaccacgcctcccgtgttggactccgacggctccttcttcctctacagcaagctcaccgtggacaagagcaggtggcagcaggggaacgtcttctcatgctccgtgatgcatgaggctctgcacaaccactacacgcagaagagcctctccctgtctcccgggaaa

SEQ ID NO: 286 - DNA, 975 bp, Artificial Sequence
  Synthetic
ggcgtgagcgacgtgccccgggatctagaagtggtggctgctacccccacaagcttgctgatctcctggacactgcctcacgctggccgggctcattactatagaattacctacggggagacaggcgggaactctcccgtgcaggaattcaccgtgcctggaaggggcgtgactgccaccatcagtgggctgaagccaggagtggactacacaattaccgtgtacgctgtgactgtgaccacaactaaagtgatccactacaaacccatctctattaattatcggaccgaaattgacaagacccacacatgcccaccttgtccagcccccgagctgctgggcggcccttcagtcttcctcttccccccaaaacccaaggacaccctcatgatctcccggacccctgaggtcacatgcgtggtggtggacgtgagccacgaagaccctgaggtcaagttcaactggtacgtggacggcgtggaggtgcataatgccaagacaaagccgcgggaggagcagtacaacagcacgtaccgtgtggtcagcgtcctcaccgtcctgcaccaggactggctgaatggcaaggagtacaagtgcaaggtctccaacaaagccctcccagcccccatcgagaaaaccatctccaaagccaaagggcagccccgagaaccacaggtgtacaccctgcccccatcccgggatgagctgaccaagaaccaggtcagcctgacctgcctggtcaaaggcttctatcccagcgacatcgccgtggagtgggagagcaatgggcagccggagaacaactacaagaccacgcctcccgtgttggactccgacggctccttcttcctctacagcaagctcaccgtggacaagagcaggtggcagcaggggaacgtcttctcatgctccgtgatgcatgaggctctgcacaaccactacacgcagaagagcctctccctgtctcccgggaaa

SEQ ID NO: 287 - DNA, 1035 bp, Artificial Sequence
  Synthetic
ggcgtgagcgacgtgccccgggatctagaagtggtggctgctacccccacaagcttgctgatctcctggacactgcctcacgctggccgggctcattactatagaattacctacggggagacaggcgggaactctcccgtgcaggaattcaccgtgcctggaaggggcgtgactgccaccatcagtgggctgaagccaggagtggactacacaattaccgtgtacgctgtgactgtgaccacaactaaagtgatccactacaaacccatctctattaattatcggaccgaaattgagtctccaaaggctcaggccagctccgtgcctaccgctcagccacaggctgagggcctggctaagacccacacatgccccccttgtccagctcccgaactgctgggcgggccttcagtcttcctcttccccccaaaacccaaggacaccctcatgatctcccggacccctgaggtcacatgcgtggtggtggacgtgagccacgaagaccctgaggtcaagttcaactggtacgtggacggcgtggaggtgcataatgccaagacaaagccgcgggaggagcagtacaacagcacgtaccgtgtggtcagcgtcctcaccgtcctgcaccaggactggctgaatggcaaggagtacaagtgcaaggtctccaacaaagccctcccagcccccatcgagaaaaccatctccaaagccaaagggcagccccgagaaccacaggtgtacaccctgcccccatcccgggatgagctgaccaagaaccaggtcagcctgacctgcctggtcaaaggcttctatcccagcgacatcgccgtggagtgggagagcaatgggcagccggagaacaactacaagaccacgcctcccgtgctggactccgacggctccttcttcctctacagcaagctcaccgtggacaagagcaggtggcagcaggggaacgtcttctcatgctccgtgatgcatgaggctctgcacaaccactacacgcagaagagcctctccctgtctcccgggaaa

SEQ ID NO: 288 - DNA, 993 bp, Artificial Sequence
  Synthetic
gacaaaactcacacatgcccaccgtgcccagcacctgaactcctggggggaccgtcagtcttcctcttccccccaaaacccaaggacaccctcatgatctcccggacccctgaggtcacatgcgtggtggtggacgtgagccacgaagaccctgaggtcaagttcaactggtacgtggacggcgtggaggtgcataatgccaagacaaagccgcgggaggagcagtacaacagcacgtaccgtgtggtcagcgtcctcaccgtcctgcaccaggactggctgaatggcaaggagtacaagtgcaaggtctccaacaaagccctcccagcccccatcgagaaaaccatctccaaagccaaagggcagccccgagaaccacaggtgtacaccctgcccccatcccgggatgagctgaccaagaaccaggtcagcctgacctgcctggtcaaaggcttctatcccagcgacatcgccgtggagtgggagagcaatgggcagccggagaacaactacaagaccacgcctcccgtgttggactccgacggctccttcttcctctacagcaagctcaccgtggacaagagcaggtggcagcaggggaacgtcttctcatgctccgtgatgcatgaggctctgcacaaccactacacgcagaagagcctctccctgtctcccggcgccggaggcggcggatccggtggcgtgtccgacgtgccccgggatctagaagtggtggctgctacccccacaagcttgctgatctcctggacactgcctcacgctggccgggctcattactatagaattacctacggggagacaggcgggaactctcccgtgcaggaattcaccgtgcctggaaggggcgtgactgccaccatcagtgggctgaagccaggagtggactacacaattaccgtgtacgctgtgactgtgaccacaactaaagtgatccactacaaacccatctctattaattatcggaccgaaatc

SEQ ID NO: 289 - DNA, 1020 bp, Artificial Sequence
  Synthetic
gacaaaactcacacatgcccaccgtgcccagcacctgaactcctggggggaccgtcagtcttcctcttccccccaaaacccaaggacaccctcatgatctcccggacccctgaggtcacatgcgtggtggtggacgtgagccacgaagaccctgaggtcaagttcaactggtacgtggacggcgtggaggtgcataatgccaagacaaagccgcgggaggagcagtacaacagcacgtaccgtgtggtcagcgtcctcaccgtcctgcaccaggactggctgaatggcaaggagtacaagtgcaaggtctccaacaaagccctcccagcccccatcgagaaaaccatctccaaagccaaagggcagccccgagaaccacaggtgtacaccctgcccccatcccgggatgagctgaccaagaaccaggtcagcctgacctgcctggtcaaaggcttctatcccagcgacatcgccgtggagtgggagagcaatgggcagccggagaacaactacaagaccacgcctcccgtgctggactccgacggctccttcttcctctacagcaagctcaccgtggacaagagcaggtggcagcaggggaacgtcttctcatgctccgtgatgcatgaggctctgcacaaccactacacgcagaagagcctctccctgtctcccgagctgcagctggaggaaagcgccgctgaggctcaggacggagaactggatggcgtgagcgacgtgccacgggatctagaagtggtggctgctacccccacaagcttgctgatctcctggacactgcctcacgctggccgggctcattactatagaattacctacggggagacaggcgggaactctcccgtgcaggaattcaccgtgcctggaaggggcgtgactgccaccatcagtgggctgaagccaggagtggactacacaattaccgtgtacgctgtgactgtgaccacaactaaagtgatccactacaaacccatctctattaattatcggaccgaaatt

SEQ ID NO: 290 - DNA, 996 bp, Artificial Sequence
  Synthetic
gacaaaactcacacatgcccaccgtgcccagcacctgaactcctggggggaccgtcagtcttcctcttccccccaaaacccaaggacaccctcatgatctcccggacccctgaggtcacatgcgtggtggtggacgtgagccacgaagaccctgaggtcaagttcaactggtacgtggacggcgtggaggtgcataatgccaagacaaagccgcgggaggagcagtacaacagcacgtaccgtgtggtcagcgtcctcaccgtcctgcaccaggactggctgaatggcaaggagtacaagtgcaaggtctccaacaaagccctcccagcccccatcgagaaaaccatctccaaagccaaagggcagccccgagaaccacaggtgtacaccctgcccccatcccgggatgagctgaccaagaaccaggtcagcctgacctgcctggtcaaaggcttctatcccagcgacatcgccgtggagtgggagagcaatgggcagccggagaacaactacaagaccacgcctcccgtgctggactccgacggctccttcttcctctacagcaagctcaccgtggacaagagcaggtggcagcaggggaacgtcttctcatgctccgtgatgcatgaggctctgcacaaccactacacgcagaagagcctctccctgtctcccggccagcccgacgagcctggcgggagcggcgtgagcgacgtgccacgggatctagaagtggtggctgctacccccacaagcttgctgatctcctggacactgcctcacgctggccgggctcattactatagaattacctacggggagacaggcgggaactctcccgtgcaggaattcaccgtgcctggaaggggcgtgactgccaccatcagtgggctgaagccaggagtggactacacaattaccgtgtacgctgtgactgtgaccacaactaaagtgatccactacaaacccatctctattaattatcggaccgaaatt

SEQ ID NO: 291 - DNA, 1008 bp, Artificial Sequence
  Synthetic
gacaaaactcacacatgcccaccgtgcccagcacctgaactcctggggggaccgtcagtcttcctcttccccccaaaacccaaggacaccctcatgatctcccggacccctgaggtcacatgcgtggtggtggacgtgagccacgaagaccctgaggtcaagttcaactggtacgtggacggcgtggaggtgcataatgccaagacaaagccgcgggaggagcagtacaacagcacgtaccgtgtggtcagcgtcctcaccgtcctgcaccaggactggctgaatggcaaggagtacaagtgcaaggtctccaacaaagccctcccagcccccatcgagaaaaccatctccaaagccaaagggcagccccgagaaccacaggtgtacaccctgcccccatcccgggatgagctgaccaagaaccaggtcagcctgacctgcctggtcaaaggcttctatcccagcgacatcgccgtggagtgggagagcaatgggcagccggagaacaactacaagaccacgcctcccgtgctggactccgacggctccttcttcctctacagcaagctcaccgtggacaagagcaggtggcagcaggggaacgtcttctcatgctccgtgatgcatgaggctctgcacaaccactacacgcagaagagcctctccctgtctcccggcggcagcgggtctggatctggcagtgggagcggctctggcgtgagcgacgtgccacgggatctagaagtggtggctgctacccccacaagcttgctgatctcctggacactgcctcacgctggccgggctcattactatagaattacctacggggagacaggcgggaactctcccgtgcaggaattcaccgtgcctggaaggggcgtgactgccaccatcagtgggctgaagccaggagtggactacacaattaccgtgtacgctgtgactgtgaccacaactaaagtgatccactacaaacccatctctattaattatcggaccgaaatt

SEQ ID NO: 292 - DNA, 917 bp, Artificial Sequence
  Synthetic
cccggacccctgaggtcacatgcgtggtggtggacgtgagccacgaagaccctgaggtcaagttcaactggtacgtggacggcgtggaggtgcataatgccaagacaaagccgcgggaggagcagtacaacagcacgtaccgtgtggtcagcgtcctcaccgtcctgcaccaggactggctgaatggcaaggagtacaagtgcaaggtctccaacaaagccctcccagcccccatcgagaaaaccatctccaaagccaaagggcagccccgagaaccacaggtgtacaccctgcccccatcccgggatgagctgaccaagaaccaggtcagcctgacctgcctggtcaaaggcttctatcccagcgacatcgccgtggagtgggagagcaatgggcagccggagaacaactacaagaccacgcctcccgtgctggactccgacggctccttcttcctctacagcaagctcaccgtggacaagagcaggtggcagcaggggaacgtcttctcatgctccgtgatgcatgaggctctgcacaaccactacacgcagaagagcctctccctgtctcccgagctgcagctggaggaaagcgccgctgaggctcaggacggagaactggatggcgtgagcgacgtgccacgggatctagaagtggtggctgctacccccacaagcttgctgatcagctgggacgctccgagaggtctggctcgatattaccgcatcacttacggcgaaacaggaggcaatagccctgtccaggagttcactgtgttcggtcgtggtaccacagctaccatcagcggccttaaacctggcgttgattataccatcactgtgtatgctgtcactatcgaccgtgacggtacccgcagcttcgacccaatttccattaattaccggaccgaaatt

SEQ ID NO: 293 - DNA, 1017 bp, Artificial Sequence
  Synthetic
gacaaaactcacacatgcccaccgtgcccagcacctgaactcctggggggaccgtcagtcttcctcttccccccaaaacccaaggacaccctcatgatctcccggacccctgaggtcacatgcgtggtggtggacgtgagccacgaagaccctgaggtcaagttcaactggtacgtggacggcgtggaggtgcataatgccaagacaaagccgcgggaggagcagtacaacagcacgtaccgtgtggtcagcgtcctcaccgtcctgcaccaggactggctgaatggcaaggagtacaagtgcaaggtctccaacaaagccctcccagcccccatcgagaaaaccatctccaaagccaaagggcagccccgagaaccacaggtgtacaccctgcccccatcccgggatgagctgaccaagaaccaggtcagcctgacctgcctggtcaaaggcttctatcccagcgacatcgccgtggagtgggagagcaatgggcagccggagaacaactacaagaccacgcctcccgtgctggactccgacggctccttcttcctctacagcaagctcaccgtggacaagagcaggtggcagcaggggaacgtcttctcatgctccgtgatgcatgaggctctgcacaaccactacacgcagaagagcctctccctgtctcccgagctgcagctggaggaaagcgccgctgaggctcaggacggagaactggatggcgtgagcgacgtgccacgggatctagaagtggtggctgctacccccacaagcttgctgatcagctgggacgctccggctggtctggctcgatattaccgcatcacttacggcgaaacaggaggcaatagccctgtccaggagttcactgtggtcggtcgtggtaacacagctaccatcagcggccttaaacctggcgttgattataccatcactgtgtatgctgtcactatcttccgtgacggtcccgtcacctgggacccaatttccattaattaccggaccgaaatt

SEQ ID NO: 294 - DNA, 1017 bp, Artificial Sequence
  Synthetic
gacaaaactcacacatgcccaccgtgcccagcacctgaactcctggggggaccgtcagtcttcctcttccccccaaaacccaaggacaccctcatgatctcccggacccctgaggtcacatgcgtggtggtggacgtgagccacgaagaccctgaggtcaagttcaactggtacgtggacggcgtggaggtgcataatgccaagacaaagccgcgggaggagcagtacaacagcacgtaccgtgtggtcagcgtcctcaccgtcctgcaccaggactggctgaatggcaaggagtacaagtgcaaggtctccaacaaagccctcccagcccccatcgagaaaaccatctccaaagccaaagggcagccccgagaaccacaggtgtacaccctgcccccatcccgggatgagctgaccaagaaccaggtcagcctgacctgcctggtcaaaggcttctatcccagcgacatcgccgtggagtgggagagcaatgggcagccggagaacaactacaagaccacgcctcccgtgctggactccgacggctccttcttcctctacagcaagctcaccgtggacaagagcaggtggcagcaggggaacgtcttctcatgctccgtgatgcatgaggctctgcacaaccactacacgcagaagagcctctccctgtctcccgagctgcagctggaggaaagcgccgctgaggctcaggacggagaactggatggcgtgagcgacgtgccacgggatctagaagtggtggctgctacccccacaagcttgctgatcagctgggacgctccgaagggtctggctcgatattaccgcatcacttacggcgaaacaggaggcaatagccctgtccaggagttcactgtggtcggtcgtggtaacacagctaccatcagcggccttaaacctggcgttgattataccatcactgtgtatgctgtcactatcttccgtgacggtcccgtcacctgggacccaatttccattaattaccggaccgaaatt

SEQ ID NO: 295 - DNA, 1020 bp, Artificial Sequence
  Synthetic
gacaaaactcacacatgcccaccgtgcccagcacctgaactcctggggggaccgtcagtcttcctcttccccccaaaacccaaggacaccctcatgatctcccggacccctgaggtcacatgcgtggtggtggacgtgagccacgaagaccctgaggtcaagttcaactggtacgtggacggcgtggaggtgcataatgccaagacaaagccgcgggaggagcagtacaacagcacgtaccgtgtggtcagcgtcctcaccgtcctgcaccaggactggctgaatggcaaggagtacaagtgcaaggtctccaacaaagccctcccagcccccatcgagaaaaccatctccaaagccaaagggcagccccgagaaccacaggtgtacaccctgcccccatcccgggatgagctgaccaagaaccaggtcagcctgacctgcctggtcaaaggcttctatcccagcgacatcgccgtggagtgggagagcaatgggcagccggagaacaactacaagaccacgcctcccgtgctggactccgacggctccttcttcctctacagcaagctcaccgtggacaagagcaggtggcagcaggggaacgtcttctcatgctccgtgatgcatgaggctctgcacaaccactacacgcagaagagcctctccctgtctcccgagctgcagctggaggaaagcgccgctgaggctcaggacggagaactggatggcgtgagcgacgtgccacgggatctagaagtggtggctgctacccccacaagcttgctgatcagctggtctctgccgaatccgggtaacgcccattattaccgcatcacttacggcgaaacaggaggcaatagccctgtccaggagttcactgtgcctggtcgtggtgttacagctaccatcagcggccttaaacctggcgttgattataccatcactgtgtatgctgtcactgttactgacacaggtttcatcacgtacaaaccaatttccattaattaccggaccgaaatt

SEQ ID NO: 296 - DNA, 1020 bp, Artificial Sequence
  Synthetic
gacaaaactcacacatgcccaccgtgcccagcacctgaactcctggggggaccgtcagtcttcctcttccccccaaaacccaaggacaccctcatgatctcccggacccctgaggtcacatgcgtggtggtggacgtgagccacgaagaccctgaggtcaagttcaactggtacgtggacggcgtggaggtgcataatgccaagacaaagccgcgggaggagcagtacaacagcacgtaccgtgtggtcagcgtcctcaccgtcctgcaccaggactggctgaatggcaaggagtacaagtgcaaggtctccaacaaagccctcccagcccccatcgagaaaaccatctccaaagccaaagggcagccccgagaaccacaggtgtacaccctgcccccatcccgggatgagctgaccaagaaccaggtcagcctgacctgcctggtcaaaggcttctatcccagcgacatcgccgtggagtgggagagcaatgggcagccggagaacaactacaagaccacgcctcccgtgctggactccgacggctccttcttcctctacagcaagctcaccgtggacaagagcaggtggcagcaggggaacgtcttctcatgctccgtgatgcatgaggctctgcacaaccactacacgcagaagagcctctccctgtctcccgagctgcagctggaggaaagcgccgctgaggctcaggacggagaactggatggcgtgagcgacgtgccacgggatctagaagtggtggctgctacccccacaagcttgctgatcagctggtctctgccgcaccaaggtaaagccaattattaccgcatcacttacggcgaaacaggaggcaatagccctgtccaggagttcactgtgcctggtcgtggtgttacagctaccatcagcggccttaaacctggcgttgattataccatcactgtgtatgctgtcactgttactgatacagggtacctcaagtacaaaccaatttccattaattaccggaccgaaatt

SEQ ID NO: 297 - DNA, 987 bp, Artificial Sequence
  Synthetic
ggcgtgagcgacgtgccccgggatctagaagtggtggctgctacccccacaagcttgctgatcagctgggacgctccgagaggtctggctcgatattaccgcatcacttacggcgaaacaggaggcaatagccctgtccaggagttcactgtgttcggtcgtggtaccacagctaccatcagcggccttaaacctggcgttgattataccatcactgtgtatgctgtcactatcgaccgtgacggtacccgcagcttcgacccaatttccattaattaccggaccgaaattgagcctaagagctccgacaaaacccacacatgcccaccttgtccagcccccgaactgctgggcggcccttcagtcttcctcttccccccaaaacccaaggacaccctcatgatctcccggacccctgaggtcacatgcgtggtggtggacgtgagccacgaagaccctgaggtcaagttcaactggtacgtggacggcgtggaggtgcataatgccaagacaaagccgcgggaggagcagtacaacagcacgtaccgtgtggtcagcgtcctcaccgtcctgcaccaggactggctgaatggcaaggagtacaagtgcaaggtctccaacaaagccctcccagcccccatcgagaaaaccatctccaaagccaaagggcagccccgagaaccacaggtgtacaccctgcccccatcccgggatgagctgaccaagaaccaggtcagcctgacctgcctggtcaaaggcttctatcccagcgacatcgccgtggagtgggagagcaatgggcagccggagaacaactacaagaccacgcctcccgtgttggactccgacggctccttcttcctctacagcaagctcaccgtggacaagagcaggtggcagcaggggaacgtcttctcatgctccgtgatgcatgaggctctgcacaaccactacacgcagaagagcctctccctgtctcccgggaaa

SEQ ID NO: 298 - DNA, 987 bp, Artificial Sequence
  Synthetic
ggcgtgagcgacgtgccccgggatctagaagtggtggctgctacccccacaagcttgctgatcagctgggacgctccggctggtctggctcgatattaccgcatcacttacggcgaaacaggaggcaatagccctgtccaggagttcactgtggtcggtcgtggtaacacagctaccatcagcggccttaaacctggcgttgattataccatcactgtgtatgctgtcactatcttccgtgacggtcccgtcacctgggacccaatttccattaattaccggaccgaaattgagcctaagagctccgacaaaacccacacatgcccaccttgtccagcccccgaactgctgggcggcccttcagtcttcctcttccccccaaaacccaaggacaccctcatgatctcccggacccctgaggtcacatgcgtggtggtggacgtgagccacgaagaccctgaggtcaagttcaactggtacgtggacggcgtggaggtgcataatgccaagacaaagccgcgggaggagcagtacaacagcacgtaccgtgtggtcagcgtcctcaccgtcctgcaccaggactggctgaatggcaaggagtacaagtgcaaggtctccaacaaagccctcccagcccccatcgagaaaaccatctccaaagccaaagggcagccccgagaaccacaggtgtacaccctgcccccatcccgggatgagctgaccaagaaccaggtcagcctgacctgcctggtcaaaggcttctatcccagcgacatcgccgtggagtgggagagcaatgggcagccggagaacaactacaagaccacgcctcccgtgttggactccgacggctccttcttcctctacagcaagctcaccgtggacaagagcaggtggcagcaggggaacgtcttctcatgctccgtgatgcatgaggctctgcacaaccactacacgcagaagagcctctccctgtctcccgggaaa

SEQ ID NO: 299 - DNA, 987 bp, Artificial Sequence
  Synthetic
ggcgtgagcgacgtgccccgggatctagaagtggtggctgctacccccacaagcttgctgatcagctgggacgctccgaagggtctggctcgatattaccgcatcacttacggcgaaacaggaggcaatagccctgtccaggagttcactgtggtcggtcgtggtaacacagctaccatcagcggccttaaacctggcgttgattataccatcactgtgtatgctgtcactatcttccgtgacggtcccgtcacctgggacccaatttccattaattaccggaccgaaattgagcctaagagctccgacaaaacccacacatgcccaccttgtccagcccccgaactgctgggcggcccttcagtcttcctcttccccccaaaacccaaggacaccctcatgatctcccggacccctgaggtcacatgcgtggtggtggacgtgagccacgaagaccctgaggtcaagttcaactggtacgtggacggcgtggaggtgcataatgccaagacaaagccgcgggaggagcagtacaacagcacgtaccgtgtggtcagcgtcctcaccgtcctgcaccaggactggctgaatggcaaggagtacaagtgcaaggtctccaacaaagccctcccagcccccatcgagaaaaccatctccaaagccaaagggcagccccgagaaccacaggtgtacaccctgcccccatcccgggatgagctgaccaagaaccaggtcagcctgacctgcctggtcaaaggcttctatcccagcgacatcgccgtggagtgggagagcaatgggcagccggagaacaactacaagaccacgcctcccgtgttggactccgacggctccttcttcctctacagcaagctcaccgtggacaagagcaggtggcagcaggggaacgtcttctcatgctccgtgatgcatgaggctctgcacaaccactacacgcagaagagcctctccctgtctcccgggaaa

SEQ ID NO: 300 - DNA, 990 bp, Artificial Sequence
  Synthetic
ggcgtgagcgacgtgccccgggatctagaagtggtggctgctacccccacaagcttgctgatcagctggtctctgccgaatccgggtaacgcccattattaccgcatcacttacggcgaaacaggaggcaatagccctgtccaggagttcactgtgcctggtcgtggtgttacagctaccatcagcggccttaaacctggcgttgattataccatcactgtgtatgctgtcactgttactgacacaggtttcatcacgtacaaaccaatttccattaattaccggaccgaaattgagcctaagagctccgacaaaacccacacatgcccaccttgtccagcccccgaactgctgggcggcccttcagtcttcctcttccccccaaaacccaaggacaccctcatgatctcccggacccctgaggtcacatgcgtggtggtggacgtgagccacgaagaccctgaggtcaagttcaactggtacgtggacggcgtggaggtgcataatgccaagacaaagccgcgggaggagcagtacaacagcacgtaccgtgtggtcagcgtcctcaccgtcctgcaccaggactggctgaatggcaaggagtacaagtgcaaggtctccaacaaagccctcccagcccccatcgagaaaaccatctccaaagccaaagggcagccccgagaaccacaggtgtacaccctgcccccatcccgggatgagctgaccaagaaccaggtcagcctgacctgcctggtcaaaggcttctatcccagcgacatcgccgtggagtgggagagcaatgggcagccggagaacaactacaagaccacgcctcccgtgttggactccgacggctccttcttcctctacagcaagctcaccgtggacaagagcaggtggcagcaggggaacgtcttctcatgctccgtgatgcatgaggctctgcacaaccactacacgcagaagagcctctccctgtctcccgggaaa

SEQ ID NO: 301 - DNA, 990 bp, Artificial Sequence
  Synthetic
ggcgtgagcgacgtgccccgggatctagaagtggtggctgctacccccacaagcttgctgatcagctggtctctgccgcaccaaggtaaagccaattattaccgcatcacttacggcgaaacaggaggcaatagccctgtccaggagttcactgtgcctggtcgtggtgttacagctaccatcagcggccttaaacctggcgttgattataccatcactgtgtatgctgtcactgttactgatacagggtacctcaagtacaaaccaatttccattaattaccggaccgaaattgagcctaagagctccgacaaaacccacacatgcccaccttgtccagcccccgaactgctgggcggcccttcagtcttcctcttccccccaaaacccaaggacaccctcatgatctcccggacccctgaggtcacatgcgtggtggtggacgtgagccacgaagaccctgaggtcaagttcaactggtacgtggacggcgtggaggtgcataatgccaagacaaagccgcgggaggagcagtacaacagcacgtaccgtgtggtcagcgtcctcaccgtcctgcaccaggactggctgaatggcaaggagtacaagtgcaaggtctccaacaaagccctcccagcccccatcgagaaaaccatctccaaagccaaagggcagccccgagaaccacaggtgtacaccctgcccccatcccgggatgagctgaccaagaaccaggtcagcctgacctgcctggtcaaaggcttctatcccagcgacatcgccgtggagtgggagagcaatgggcagccggagaacaactacaagaccacgcctcccgtgttggactccgacggctccttcttcctctacagcaagctcaccgtggacaagagcaggtggcagcaggggaacgtcttctcatgctccgtgatgcatgaggctctgcacaaccactacacgcagaagagcctctccctgtctcccgggaaa

SEQ ID NO: 302 - DNA, 1020 bp, Artificial Sequence
  Synthetic
gacaaaactcacacatgcccaccgtgcccagcacctgaactcctggggggaccgtcagtcttcctcttccccccaaaacccaaggacaccctcatgatctcccggacccctgaggtcacatgcgtggtggtggacgtgagccacgaagaccctgaggtcaagttcaactggtacgtggacggcgtggaggtgcataatgccaagacaaagccgcgggaggagcagtacaacagcacgtaccgtgtggtcagcgtcctcaccgtcctgcaccaggactggctgaatggcaaggagtacaagtgcaaggtctccaacaaagccctcccagcccccatcgagaaaaccatctccaaagccaaagggcagccccgagaaccacaggtgtacaccctgcccccatcccgggatgagctgaccaagaaccaggtcagcctgacctgcctggtcaaaggcttctatcccagcgacatcgccgtggagtgggagagcaatgggcagccggagaacaactacaagaccacgcctcccgtgctggactccgacggctccttcttcctctacagcaagctcaccgtggacaagagcaggtggcagcaggggaacgtcttctcatgctccgtgatgcatgaggctctgcacaaccactacacgcagaagagcctctccctgtctcccgagctgcagctggaggaaagcgccgctgaggctcaggaaggagaactggaaggcgtgagcgacgtgccacgggatctagaagtggtggctgctacccccacaagcttgctgatctcctggacactgcctcacgctggccgggctcattactatagaattacctacggggagacaggcgggaactctcccgtgcaggaattcaccgtgcctggaaggggcgtgactgccaccatcagtgggctgaagccaggagtggactacacaattaccgtgtacgctgtgactgtgaccacaactaaagtgatccactacaaacccatctctattaattatcggaccgaaatt

SEQ ID NO: 303 - DNA, 1017 bp, Artificial Sequence
  Synthetic
gacaaaactcacacatgcccaccgtgcccagcacctgaactcctggggggaccgtcagtcttcctcttccccccaaaacccaaggacaccctcatgatctcccggacccctgaggtcacatgcgtggtggtggacgtgagccacgaagaccctgaggtcaagttcaactggtacgtggacggcgtggaggtgcataatgccaagacaaagccgcgggaggagcagtacaacagcacgtaccgtgtggtcagcgtcctcaccgtcctgcaccaggactggctgaatggcaaggagtacaagtgcaaggtctccaacaaagccctcccagcccccatcgagaaaaccatctccaaagccaaagggcagccccgagaaccacaggtgtacaccctgcccccatcccgggatgagctgaccaagaaccaggtcagcctgacctgcctggtcaaaggcttctatcccagcgacatcgccgtggagtgggagagcaatgggcagccggagaacaactacaagaccacgcctcccgtgctggactccgacggctccttcttcctctacagcaagctcaccgtggacaagagcaggtggcagcaggggaacgtcttctcatgctccgtgatgcatgaggctctgcacaaccactacacgcagaagagcctctccctgtctcccgagctgcagctggaggaaagcgccgctgaggctcaggaaggagaactggaaggcgtgagcgacgtgccacgggatctagaagtggtggctgctacccccacaagcttgctgatcagctgggacgctccggctggtctggctcgatattaccgcatcacttacggcgaaacaggaggcaatagccctgtccaggagttcactgtggtcggtcgtggtaacacagctaccatcagcggccttaaacctggcgttgattataccatcactgtgtatgctgtcactatcttccgtgacggtcccgtcacctgggacccaatttccattaattaccggaccgaaatt

SEQ ID NO: 304 - DNA, 1017 bp, Artificial Sequence
  Synthetic
gacaaaactcacacatgcccaccgtgcccagcacctgaactcctggggggaccgtcagtcttcctcttccccccaaaacccaaggacaccctcatgatctcccggacccctgaggtcacatgcgtggtggtggacgtgagccacgaagaccctgaggtcaagttcaactggtacgtggacggcgtggaggtgcataatgccaagacaaagccgcgggaggagcagtacaacagcacgtaccgtgtggtcagcgtcctcaccgtcctgcaccaggactggctgaatggcaaggagtacaagtgcaaggtctccaacaaagccctcccagcccccatcgagaaaaccatctccaaagccaaagggcagccccgagaaccacaggtgtacaccctgcccccatcccgggatgagctgaccaagaaccaggtcagcctgacctgcctggtcaaaggcttctatcccagcgacatcgccgtggagtgggagagcaatgggcagccggagaacaactacaagaccacgcctcccgtgctggactccgacggctccttcttcctctacagcaagctcaccgtggacaagagcaggtggcagcaggggaacgtcttctcatgctccgtgatgcatgaggctctgcacaaccactacacgcagaagagcctctccctgtctcccgagctgcagctggaggaaagcgccgctgaggctcaggaaggagaactggaaggcgtgagcgacgtgccacgggatctagaagtggtggctgctacccccacaagcttgctgatcagctgggacgctccgaagggtctggctcgatattaccgcatcacttacggcgaaacaggaggcaatagccctgtccaggagttcactgtggtcggtcgtggtaacacagctaccatcagcggccttaaacctggcgttgattataccatcactgtgtatgctgtcactatcttccgtgacggtcccgtcacctgggacccaatttccattaattaccggaccgaaatt

SEQ ID NO: 305 - DNA, 1020 bp, Artificial Sequence
  Synthetic
gacaaaactcacacatgcccaccgtgcccagcacctgaactcctggggggaccgtcagtcttcctcttccccccaaaacccaaggacaccctcatgatctcccggacccctgaggtcacatgcgtggtggtggacgtgagccacgaagaccctgaggtcaagttcaactggtacgtggacggcgtggaggtgcataatgccaagacaaagccgcgggaggagcagtacaacagcacgtaccgtgtggtcagcgtcctcaccgtcctgcaccaggactggctgaatggcaaggagtacaagtgcaaggtctccaacaaagccctcccagcccccatcgagaaaaccatctccaaagccaaagggcagccccgagaaccacaggtgtacaccctgcccccatcccgggatgagctgaccaagaaccaggtcagcctgacctgcctggtcaaaggcttctatcccagcgacatcgccgtggagtgggagagcaatgggcagccggagaacaactacaagaccacgcctcccgtgctggactccgacggctccttcttcctctacagcaagctcaccgtggacaagagcaggtggcagcaggggaacgtcttctcatgctccgtgatgcatgaggctctgcacaaccactacacgcagaagagcctctccctgtctcccgagctgcagctggaggaaagcgccgctgaggctcaggaaggagaactggaaggcgtgagcgacgtgccacgggatctagaagtggtggctgctacccccacaagcttgctgatcagctggtctctgccgcaccaaggtaaagccaattattaccgcatcacttacggcgaaacaggaggcaatagccctgtccaggagttcactgtgcctggtcgtggtgttacagctaccatcagcggccttaaacctggcgttgattataccatcactgtgtatgctgtcactgttactgatacagggtacctcaagtacaaaccaatttccattaattaccggaccgaaatt

SEQ ID NO: 306 - protein, 10 aa, Artificial Sequence
  Synthetic
MGVSDVPRDL

SEQ ID NO: 307 - protein, 9 aa, Artificial Sequence
  Synthetic
GVSDVPRDL

SEQ ID NO: 308 - protein, 8 aa, Artificial Sequence
  Synthetic
VSDVPRDL

SEQ ID NO: 309 - protein, 7 aa, Artificial Sequence
  Synthetic
SDVPRDL

SEQ ID NO: 310 - protein, 6 aa, Artificial Sequence
  Synthetic
DVPRDL

SEQ ID NO: 311 - protein, 5 aa, Artificial Sequence
  Synthetic
VPRDL

SEQ ID NO: 312 - protein, 4 aa, Artificial Sequence
  Synthetic
PRDL

SEQ ID NO: 313 - protein, 7 aa, Artificial Sequence
  Synthetic
EIEPKSS

SEQ ID NO: 314 - protein, 6 aa, Artificial Sequence
  Synthetic
EIDKPC

SEQ ID NO: 315 - protein, 5 aa, Artificial Sequence
  Synthetic
EIDKP

SEQ ID NO: 316 - protein, 4 aa, Artificial Sequence
  Synthetic
EIDK

SEQ ID NO: 317 - protein, 6 aa, Artificial Sequence
  Synthetic
EIDKPS

SEQ ID NO: 318 - protein, 7 aa, Artificial Sequence
  Synthetic
EIEKPSQ

SEQ ID NO: 319 - protein, 9 aa, Artificial Sequence
  Synthetic
EIDKPSQLE

SEQ ID NO: 320 - protein, 12 aa, Artificial Sequence
  Synthetic
EIEDEDEDEDED

SEQ ID NO: 321 - protein, 5 aa, Artificial Sequence
  Synthetic
EGSGS

SEQ ID NO: 322 - protein, 7 aa, Artificial Sequence
  Synthetic
EIDKPCQ

SEQ ID NO: 323 - protein, 5 aa, Artificial Sequence
  Synthetic
EGSGC

SEQ ID NO: 324 - protein, 9 aa, Artificial Sequence
  Synthetic
EIDKPCQLE

SEQ ID NO: 325 - protein, 13 aa, Artificial Sequence
  Synthetic
EIDKPSQHHHHHH

SEQ ID NO: 326 - protein, 10 aa, Artificial Sequence
  Synthetic
GSGCHHHHHH

SEQ ID NO: 327 - protein, 11 aa, Artificial Sequence
  Synthetic
EGSGCHHHHHH

SEQ ID NO: 328 - protein, 6 aa, Artificial Sequence
  Synthetic
HHHHHH

SEQ ID NO: 329 - protein, 17 aa, Artificial Sequence
  Synthetic
LYFNGKEQIIYGKIPAM

SEQ ID NO: 330 - protein, 11 aa, Artificial Sequence
  Synthetic
PHTHLVHQANP

SEQ ID NO: 331 - protein, 87 aa, Artificial Sequence
  Synthetic
EVVAATPTSLLISWSLPHQGKANYYRITYGETGGNSPVQEFTVPGRGVTATISGLKPGVDYTITVYAVTVTDTGYLKYKPISINYRT